European Patent Specification EP 3 752 608 B1, published March 18, 2026. Title: GENE THERAPY. Applicant: UCL Business PLC. The sequence listing filed with the application follows.

SEQUENCE LISTING (41 sequences)

SEQ ID NO: 1 - DNA, 2105 bp, Homo sapiens
tccgggttttgcggcggagcgggcgggctgcgcgtgcggcggcttcaactgtcgcggtaggcagcagcaggctgaagggatcatggtgcagtacgagctgtgggccgcgctgcctggcgcctccggggtcgccctggcctgctgcttcgtggcggcggccgtggccctgcgctggtccgggcgccggacggcgcggggcgcggtggtccgggcgcgacagaggcagcgagcgggcctggagaacatggacagggcggcgcagcgcttccggctccagaacccagacctggactcagaggcgctgctagccctgcccctgcctcagctggtgcagaagttacacagtagagagctggcccctgaggccgtgctcttcacctatgtgggaaaggcctgggaagtgaacaaagggaccaactgtgtgacctcctatctggctgactgtgagactcagctgtctcaggccccaaggcagggcctgctctatggcgtccctgtgagcctcaaggagtgcttcacctacaagggccaggactccacgctgggcttgagcctgaatgaaggggtgccggcggagtgcgacagcgtagtggtgcatgtgctgaagctgcagggtgccgtgcccttcgtgcacaccaatgttccacagtccatgttcagctatgactgcagtaaccccctctttggccagaccgtgaacccatggaagtcctccaaaagcccagggggctcctcagggggtgaaggggccctcatcgggtctggaggctcccccctgggcttaggcactgatatcggaggcagcatccgcttcccctcctccttctgcggcatctgcggcctcaagcccacagggaaccgcctcagcaagagtggcctgaagggctgtgtctatggacaggaggcagtgcgtctctccgtgggccccatggcccgggacgtggagagcctggcactgtgcctgcgagccctgctgtgcgaggacatgttccgcttggaccccactgtgcctcccttgcccttcagagaagaggtctacaccagctctcagcccctgcgtgtggggtactatgagactgacaactataccatgccctccccggccatgaggcgggccgtgctggagaccaaacagagccttgaggctgcggggcacacgctggttcccttcttgccaagcaacataccccatgctctggagaccctgtcaacaggtgggctcttcagtgatggtggccacaccttcctacagaacttcaaaggtgatttcgtggacccctgcctgggggacctggtctcaattctgaagcttccccaatggcttaaaggactgctggccttcctggtgaagcctctgctgccaaggctgtcagctttcctcagcaacatgaagtctcgttcggctggaaaactctgggaactgcagcacgagatcgaggtgtaccgcaaaaccgtgattgcccagtggagggcgctggacctggatgtggtgctgacccccatgctggcccctgctctggacttgaatgccccaggcagggccacaggggccgtcagctacactatgctgtacaactgcctggacttccctgcaggggtggtgcctgtcaccacggtgactgctgaggacgaggcccagatggaacattacaggggctactttggggatatctgggacaagatgctgcagaagggcatgaagaagagtgtggggctgccggtggccgtgcagtgtgtggctctgccctggcaagaagagttgtgtctgcggttcatgcgggaggtggagcgactgatgacccctgaaaagcagtcatcctgatggctctggctccagaggacctgagactcacactctctgcagcccagcctagtcagggcacagctgccctgctgccacagcaaggaaatgtcctgcatggggcagaggcttccgtgtcctctcccccaaccccctgcaagaagcgccgactccctgagtctggacctccatccctgctctggtcccctctcttcgtcctgatccctccacccccatgtggcagcccatgggtatgacataggccaaggcccaactaacagtcaagaaacagctaaaaaaaaaa

SEQ ID NO: 2 - DNA, 2105 bp, Homo sapiens
tccgggttttgcggcggagcgggcgggctgcgcgtgcggcggcttcaactgtcgcggtaggcagcagcaggctgaagggatcatggtgcagtacgagctgtgggccgcgctgcctggcgcctccggggtcgccctggcctgctgcttcgtggcggcggccgtggccctgcgctggtccgggcgccggacggcgcggggcgcggtggtccgggcgcgacagaggcagcgagcgggcctggagaacatggacagggcggcgcagcgcttccggctccagaacccagacctggactcagaggcgctgctagccctgcccctgcctcagctggtgcagaagttacacagtagagagctggcccctgaggccgtgctcttcacctatgtgggaaaggcctgggaagtgaacaaagggaccaactgtgtgacctcctatctggctgactgtgagactcagctgtctcaggccacaaggcagggcctgctctatggcgtccctgtgagcctcaaggagtgcttcacctacaagggccaggactccacgctgggcttgagcctgaatgaaggggtgccggcggagtgcgacagcgtagtggtgcatgtgctgaagctgcagggtgccgtgcccttcgtgcacaccaatgttccacagtccatgttcagctatgactgcagtaaccccctctttggccagaccgtgaacccatggaagtcctccaaaagcccagggggctcctcagggggtgaaggggccctcatcgggtctggaggctcccccctgggcttaggcactgatatcggaggcagcatccgcttcccctcctccttctgcggcatctgcggcctcaagcccacagggaaccgcctcagcaagagtggcctgaagggctgtgtctatggacaggaggcagtgcgtctctccgtgggccccatggcccgggacgtggagagcctggcactgtgcctgcgagccctgctgtgcgaggacatgttccgcttggaccccactgtgcctcccttgcccttcagagaagaggtctacaccagctctcagcccctgcgtgtggggtactatgagactgacaactataccatgccctccccggccatgaggcgggccgtgctggagaccaaacagagccttgaggctgcggggcacacgctggttcccttcttgccaagcaacataccccatgctctggagaccctgtcaacaggtgggctcttcagtgatggtggccacaccttcctacagaacttcaaaggtgatttcgtggacccctgcctgggggacctggtctcaattctgaagcttccccaatggcttaaaggactgctggccttcctggtgaagcctctgctgccaaggctgtcagctttcctcagcaacatgaagtctcgttcggctggaaaactctgggaactgcagcacgagatcgaggtgtaccgcaaaaccgtgattgcccagtggagggcgctggacctggatgtggtgctgacccccatgctggcccctgctctggacttgaatgccccaggcagggccacaggggccgtcagctacactatgctgtacaactgcctggacttccctgcaggggtggtgcctgtcaccacggtgactgctgaggacgaggcccagatggaacattacaggggctactttggggatatctgggacaagatgctgcagaagggcatgaagaagagtgtggggctgccggtggccgtgcagtgtgtggctctgccctggcaagaagagttgtgtctgcggttcatgcgggaggtggagcgactgatgacccctgaaaagcagtcatcctgatggctctggctccagaggacctgagactcacactctctgcagcccagcctagtcagggcacagctgccctgctgccacagcaaggaaatgtcctgcatggggcagaggcttccgtgtcctctcccccaaccccctgcaagaagcgccgactccctgagtctggacctccatccctgctctggtcccctctcttcgtcctgatccctccacccccatgtggcagcccatgggtatgacataggccaaggcccaactaacagtcaagaaacagctaaaaaaaaaa

SEQ ID NO: 3 - DNA, 2845 bp, Homo sapiens
ggcaaaggcgccattctcctgggtacagtgacttgcagtctcagtgatgaccattgagatggagactggatggaggcccctgaggagagcagaatggttcccacatcagggcccctctgcaccacttttccagtctcctcatgtcttctctgttcctcgtctgggaagtcatctcccttacccccacaactcccctccaccagcagggagagtcaatagactggggaggctggaaccccagatcagagtcatggccttgctttggagtcaagggggaagcccagctgggcgggctggtctcatgtcctggcatcatctcccctggggtggatgcctgatgagccctgcccgctcctccaggtgttctttcctttcctctcttcctgtcccccagaacctccactctaggcaaacatggcctgttcagttccacctccatgcgtctgcttatgcggaacaaaggagctttgggagaatcctgaaggcaatgggaaccccaggagcaaccccatccataactcctgagggttggagtagggaatctgaggggtgggatctgagaggtaggatgggtgggagtaggatgtgacagaggtgaggtcagctgcccagctgcaggcttgggcccttcttcaggctcgcctgctaaagcctcttcctctgcatggcccgggagataggggttttgtcgccaggaagtccagatggggtaagaactaggaggaggttgatcactgccacacccagggcccgagatgtgcgtgggtgccctggcagcatcgctgacaaatactcctgaggaaacagcagctggattcacacaggtcgtgcaatacctaaggtggcttggctgtttgactccctgatgatgctacttctgctggccctgctgggggctggcctactgggggcttccctgctcacctcgtggcatgctccagcccggaacaagatccccagggcccagaagtggagggaggtagcactgcagaagatggaggacctggcccagtgactccggcagcagacggagtctcactttgttgcccaggctggagtgcagtggcctgatctcagctccctgcaacctccacctcccgagttgaagcaattctcttgcctcagcctccagagtagctgggattacaggagccagatctggaccccaagccaatcctggagctgcccctggcagagctggcccagcagcttcggaccgaagagctgagtctggagagcatcctctgtagctacttaaagcaggcactgaaggtgcaccaggaggtgaactgcctgatggatttcctgggggaatgtgaggaggaactgcaggcattaaagaagcttaagaagagtgagagaggccttctctatggggtccccatgagcctcaaggacacctatgacagcatgggccatgactgtgcatgccgcctggcctagttcctggagaagcctgcgaccaaggacggggtcattatgaaagtgctcaaggcccaaggagccatcccctttgttaagaccaacatcccactgacgctgctcagctttgaatgcggcaactcccatctatggccagatgttgagcccactgaacttaaagaagacatgtgggggctcctcagggggtgaggggctctgctggcagaaagggggtccatcctaggcatgggtactgacacaggtgacagcatctgcataccagccagcttctgtggtgtttatggcctctggaccacaggttcccgcctcagctacactggaattgcctctgccatcaaggggaaaaaaatcggtgaccacggtggctggccccatggcccaggacgtggagagcctggcgctgtgcctgcaagccctgctgagtgaagacatgtaccgactggaccccactgtgctccagatgccctttagggaggaggtgaagaccccctttcccaccccaggctgcagtgagtgagaagcccacatgctcagtccagtttgtttccttcccctgctggacaccagctgctttggcttcttggctatctggagccatagcttgacacccaagaaactgtgggaacagcacacagcagtggaggaatatgagcaagagttcatagccaagtggaggtccctggacctggatgtgctgctggtgccagttctgggctctgccttctatataggctcttcctccctagcatcagaaagtcagtcttatgtgaccctgtacaacctcctggactttcccgcgggcgtggtgcctgtcactatcgtgacactacaggacgaggaggaactggccttctacaaggggtgctacggagatagttctgacaaaaatttctcagaggcggtaagaggatccgtcggacttctggtgactgtgcagtgcattgctttgccatgggaagaggagctgtgtctccggttcatgaaggaggtggacaccttggtcaagaatcagagggggcccaagtgataggctcctggaatggagtaacagctcatgaaacacggggctggttgtggtggctcatacttgtaatcccagcagttcaggaggcagaggctggcagatcgcttgaggccacgagtttgagaccaacctgggcaacatagtgagaccctgcttctaaagcattttcttggtgttactcctgtagatcctcacccaagtgtgctcctgatgccccttccttctcatgaataccatgtccaccttatgtctcctccttctggaaccccaccaggttccttttctttgttggtccctctgtgtgggtgctcaatattcctcagatgggcccaggatggggagcagggtgaggagctcaataaacattttctgactggc

SEQ ID NO: 4 - DNA, 1696 bp, Homo sapiens
gagccagatctggaccccaagccaatcctggagctgcccctggcagagctggcccagcagcttcggaccgaagagctgagtctggagagcatcctctgtagctacttaaagcaggcactgaaggtgcaccaggaggtgaactgcctgatggatttcctgggggaatgtgaggaggaactgcaggcattaaagaagcttaagaagagtgagagaggccttctctatggggtccccatgagcctcaaggacacctatgacagcatgggccatgactgtgcatgccgcctggcctagttcctggagaagcctgcgaccaaggacggggtcattatgaaagtgctcaaggcccaaggagccatcccctttgttaagaccaacatcccactgacgctgctcagctttgaatgcggcaactcccatctatggccagatgttgagcccactgaacttaaagaagacatgtgggggctcctcagggggtgaggggctctgctggcagaaagggggtccatcctaggcatgggtactgacacaggtgacagcatctgcataccagccagcttctgtggtgtttatggcctctggaccacaggttcccgcctcagctacactggaattgcctctgccatcaaggggaaaaaaatcggtgaccacggtggctggccccatggcccaggacgtggagagcctggcgctgtgcctgcaagccctgctgagtgaagacatgtaccgactggaccccactgtgctccagatgccctttagggaggaggtgaagaccccctttcccaccccaggctgcagtgagtgagaagcccacatgctcagtccagtttgtttccttcccctgctggacaccagctgctttggcttcttggctatctggagccatagcttgacacccaagaaactgtgggaacagcacacagcagtggaggaatatgagcaagagttcatagccaagtggaggtccctggacctggatgtgctgctggtgccagttctgggctctgccttctatataggctcttcctccctagcatcagaaagtcagtcttatgtgaccctgtacaacctcctggactttcccgcgggcgtggtgcctgtcactatcgtgacactacaggacgaggaggaactggccttctacaaggggtgctacggagatagttctgacaaaaatttctcagaggcggtaagaggatccgtcggacttctggtgactgtgcagtgcattgctttgccatgggaagaggagctgtgtctccggttcatgaaggaggtggacaccttggtcaagaatcagagggggcccaagtgataggctcctggaatggagtaacagctcatgaaacacggggctggttgtggtggctcatacttgtaatcccagcagttcaggaggcagaggctggcagatcgcttgaggccacgagtttgagaccaacctgggcaacatagtgagaccctgcttctaaagcattttcttggtgttactcctgtagatcctcacccaagtgtgctcctgatgccccttccttctcatgaataccatgtccaccttatgtctcctccttctggaaccccaccaggttccttttctttgttggtccctctgtgtgggtgctcaatattcctcagatgggcccaggatggggagcagggtgaggagctcaataaacattttctgactggc

SEQ ID NO: 5 - DNA, 26960 bp, Homo sapiens
tttcgctcttgttgtgcaggctggagtgcaatggcgagatctcagctcactgcaacctctgcctaccggattcaagtgattctcctgcctcagcctcccgagtatctgggattacaggcgtgtgccaccatgcccagctaattttgtatttttagtagagatgggatttctccatgttagtcaggctggtcttgaactcctgacctcaggtgatctgcctgccttggcctcccaaagtgctgggattacaggcgtgagccactgtgcccggcctgccacagctttttgcctcgcttccctgggctccagactggacatctccaacaatctttcacatggcagttaggcaatctcatgcttaaaatctttggactcacttgtgccaagtccagaagccttgttatgacctgcaaggccatgattaacctgaccctgcagctggcccctgcggcctcatctcctgcccttcctcagtgctcacagcccggccacgtggcctgcaggtaatgttcagaacaccgagtgatctcccgcctccacgccctttgctcttggtgcttgctgtgcctggagtgttgttcctggggtctccacctaaagaccacctactcgtccaaggtgagggcaattgctcttccaactctgtcaggctgtgttgaaagagcttctttgtgcttctgcacgtggtcaaaagcaaggtctgtgtattaatagaacccaacatctgttaggctgtggagttgaatacccattatctcatttggaaagtgggcattactatttccatttaaaaaatttatttatttatttattttttgagacagagtctctctctgtcgcccaggctggagttcaatggcacgatcttggctcactgcaacctctgtctctgggttcaagtgattctcctgcctcagcctcccaagtagctgggattacaggcgcctgccactgtgcccggctatgttttgtatttgtagtagagatggggtttcaccacgttggccaggctggtttcgaactcccgacctcaggtggtccacctgccttggccaaagtgctgggattacaggcgtgagccactgcgcctggccttttttcttttctttttctttgagatggcgtcttcctctgccacccaggctggagtgcagtggtgcgatctcagctcactgcagcctccgcctcctggcttcaagcgattttcctgcctcagactcccgagtatagctgggactccaggcgcctgccaccatgcctggctatgttttgtatttgtggtagagatggggtttcactatgttggccaggctggtcctcaactcctgatctcaagtgatccgcccgccttggcctcccaaagtgctgagattacaggtgtgagctaccgtgtctggccctattatttccattttatacataaggaaactgaagttcagaggggattgctgacttgttgaaggctgatcattatgggttacagagaagacttgaaacccacacgctcaactctaaacttactgtgacttcctcatttgtacaatcatcacaagaacatgcattcaacattcttcggacaccagcctctgtgctaggcgaccacaacactttgaagacagaagcagtcctgtgtactgtgcacctctgccaatatctgtttacaggagatagctgccatgtccctgtccaccctcccttttctctcctggcgattgcgatattggagttttaggacacagccagagcacttgtcatttgttcctgttggacaccatttttaggattatcccaagagctctggctgtttctgctcttcctcccaacatgtgcttatccacaaatctgagcactggacctctgcaacttcatccaagtcacccataaacctatggatcacagcagaccaaggaaagggcgtgacctacacccttaacagacagacacataaccgagttttgagcttcccagccagatgtatctttagttcacatttctctggctgggcttagctgggccctcccaagtttcctacacatagatttggggtggcggccctgggcacctcaggaaggtgaagccacttgggatcgggctgtgtatgctcagcacccagcatggtgcctggtactcagtgggtacccagagaaggcttgttgaatggagcaatgggtgacttgttattagggaacccattttggtccattctgattacttcctcttctcacctccaatagggaattttccaatcagtccctgaccctttgctcctttcacatttattgtatctacctccatgatcttttttttttttttttttgagatggagtcttgcactgttgcccaggctggagtgcaatggcaggatctcggcttactgcaacctctgcctcctgggttcaagcgattttcctgcctcagcctccggagtagctgggattataggcgcctgccaccacgcccagctaattttttgtatttatagtagagatggggtttcactatgttggctaggctggtctcgaactcttgacctcaggcaatccacctgcctcagcctcccaaaatgctaggagccatgatcttgattagtgcccatgaggacaaataattcccagtctacattcaacctatagctttctcctggtctgtagatcctcatctatccacttctctcatcctcttaactccttcatctctctcaggctgttgaaagagcttctttgtgcttctgcacttggtagaaagcagggactgtgtcttaatagaatccaacatccgttaggctgtggagttgaacccattatctcctttgtaaaatgggcttattatttccatttcatatataaggaaactgaaattcagagagggttgctctctgaacaacaatggagggttgctccctccattcatcctcccatccatgcaataaaaatattgaattcttcccacagtatgttcagggtaaccaatcagaaatagtccctgcctgaatggagcttccattctaccaggaaacagacatcaaatgtagaattacacagaaacactcgttagaagtgcaatcaagcagaagccctgggtattatgagaataaaccacgtgggatctgatccagcctgagatgtgtgtatgtgtgtgtcagggaatgcttcctggaggaagtaacattgaagctgaaaactgcattgtcacctgagccaaggaatgagtgtgtttcaaggagggtgaagctgacaactctaaatgctgctgatttactcttgaggagatcactgggatgatataggcacaagccagactttgttgggtgggggagtgagtgaaaggtgaagaagtaaaggcagcccgtgtagaaaactggaaaagttcaggaagcggacaaaagacgtggtagtagttagggagggtgtaaatctgagggaatcatccctcatcccccaagataggagagacttagcatgttaaatgctgctaggaaagagctagcagcaacgcacagaggggggaagtcaaggtaggaatggagggctcaacctgccatcatttcttcactgaagagataccattgaacacataccatgtgccaggtgttttgaaaaaggctgacaaggtctatgctcccccaaccccccagctaatttttttgcattttctgtagagatggggtcttgccgtgttgtccaggttgagctcaaactcctgagctcaattgatccgcccaaagtgctgggattacaggcgtgagccactgtgcctggcctcgtctgtgcttttacggagcttattttctagggagggaggcaggaggtgagttacagatcaacaagaaaacttcagctaatgataagtgtaatgatgagataaaatgaggtatgtggtaacggaagggtgtaacccaggaaaaggtgaggtcacgaggcctagagtgctgtgccgtgggatgtggtgcgggtgacaagtggcctgggggagctgaagatatgggggagagctggagttcatgaaggtggagtgggggctatggaagaaaatggtcagaaaagaggcagaaggacagaggagggctggtctggaggccccagggagatgacagagtgttacagagtgggcaacttcagggtcacccttagtcaactgctgacctcgcatctgttcctttagaccctcgggtactcagactcaacattaccaaccatgaattcagttccttcccaccctaacctgctgctgccctggcttcctggtctggagggcaaaggcgccattctcctgggtacagtgacttgcagtctcagtgatgaccattgagatggagactggatggaggcccctgaggagagcagaatggttcccacatcagggcccctctgcaccacttttccagtctcctcatgtcttctctgttcctcgtctgggaagtcatctcccttacccccacaactcccctccaccagcagggagagtcaatagactggggaggctggaaccccggatcagagtcatggccttgctttggagtcaagggggaagcccagctgggcgggctggtctcatgtcctggcatcatctcccctggggtggatgcctgatgagccctgcccgctcctccaggtgttctttcctttcctctcttcctgtcccccagaacctccactctaggcaaacatggcctgttcagttccacctccatgcgtctgcttatgcggaacaaaggagctttgggagaatcctgaaggcaatgggaaccccaggagcaaccccatccataactcctgagggttggagtagggaatctgaggggtgggatctgagaggtaggatgggtgggagtaggatgtgacagaggtgaggtcagctgcccagctgcaggcttgggcccttcttcaggctcgcctgctaaagcctcttcctctgcatggcccgggagataggggttttgtcgccaggaagtccagatggggtaagaactaggaggaggttgatcactgccacacccagggcccgagatgtgcgtgggtgccctggcagcatcgctgacaaatactcctgaggaaacagcagctggattcacacaggtcgtgcaatacctaaggtggcttggctgtttgactccctgatgatgctacttctgctggccctgctgggggctggcctactgggggcttccctgctcacctcgtggcatgctccagcccggaacaagatccccagggcccagaagtggagggaggtagcactgcagaagatggaggacctggcccagtgactccggcagcaggtgagtcgacacgggtcccggaggcccccagccacagggggccttggccctcaatcccaacaggaggactacacctcaggatgcccctcccgtccatgaccccagcccccgcagacacagggagcaggtgggcacttccccacccccagttctccccccatgccagctctgtgtgtggttgtcagttctcctccatccccggcctttgagaccctggagattgggggcagtgtattctttctctgttctcccagcacttggcacgtggctcagtaacatgggaggtgcccacttagggtatttgcggaaataagataaactgatggaggccattggaggagggaggctcgatctcttttagcccctgagcactccaaaatcccccaagacaggaaccctagtctacctgtcccctcctacctccaccccattcagctctgaaaacacttgctgagccctgataagtgcagagcatggggggctggggatggggtctcccaggaagctgcaggtcttcagaggcagctttggcaactcggagtgggggtatttcactgggatagcctctgtggctggctgggctgagactggcaggcgaagtggctgagccatagatgtatcagcaaagcctgccccaggtggcagagagaagggcgggaaggagggacatggagacaaacatagactgagcctgggatttgctgtgtggcctggaggatgtgacaacccgtctctgggccttggactccccagctgtctgaggggggatgggctcatggtctctcggggtctccagctttggttgatgatggtggactcagtctgggagcccggaggtaggggctggggctagtgcctgaggtgctgttcccatgctttggagttcctgagtgtcctctgctgtcccctggatggtgattgatggccccaatgggcagcttctctgtctgagttgctgcagttgctgagtatgtgtattaatattaattagggctaattagttggataaatcaatctgcccccagagagcagctgcccctccctggttgatgaggaggaagtctgggctaatgggttgcagtggtgaatgggcatgatggaggcgtcctgtgtgcgtgtggaggccccatctgtgtgcggtggtgggtatagcttcctttactgcggacgagggcctgctttcttgtgcctcctgctggcatttcattgtgttgtggttggttgtgtgtctggtctggctgtgtggttatgtgcctggctgggtgtgcatgtgttgggttattggttggagtgtgtacatctagctatgtgtggctggtgtgggtctgaatgtctggtagagagtgtttgtgtgtggttgtgtgtctgatgtgtgggggcagctggtttggtatgtgtctgggcatctggttggtgaacatgtggatgtctgggctgttgggctggggacctggagggggtatatgtctggatggctggaggagtggaagaggttttggggtgaggtcactcatggtgtctccagcctcccattgtggtttcaggcttcttggctctcagcaccttgctgtctccccaacaagctatacaggtctgtcctgggcaccttctcagtcatgtcaccctctctctgccagtgacaacctcgagacctcaggtgtccacctttatgtcccggggaggtgcaaggctgggacacaggtcaaaccctcacaggctcagcaaacaaattcaattctgctgagtttagtaaaatttcccagggaatttctccaggtcttgccctgtgctgagctctggggacacattcattataaagatgaatctgacccctgactcacacttgtgctaaaaatgttcccaacctgggaggggcgtggtggagatagagctgtgcagactatgcagggcagcagcacggcagagtgtggtgaggccagatgcccacagaactggtgacttggcaggagggtggctggtctgtctggagaggatcatgttgggagggctccccagacgggtggtgagtgagctgaacctcatggcacctgtaggacttttctgaaaggagaaacgagaaaggcagtaccagggagggagaagccccagatgaggcagtgtttctgtagaacgtatagaaaataatattcctaggacccattgggtaaatggaccagctgctcatggctggaactgctcaagctactcatggccaggaagctctgctcacctcaggcagagcctggccaccttgagagttgacggtttttatgatactaaacatttaaccaccacattggaatttttttttttttcagacggagtctcactttgttgcccaggctggagtgcagtggcctgatctcagctccctgcaacctccacctcccgagttgaagcaattctcttgcctcagcctccagagtagctgggattacaggcaagtcccaccaagcccaactaatttttgtatttttcgtagacatggggtttcaccatgttggccaggatggtcttgatctcttgacctcgtgatcctcccaccttggcctcccaaagtgctgggattacaggcgtgagccaccgtgcccggccataaatattaataatacattgattcactaaaaactttaaattacattttttttgtttttcaaactaggctggaggcagcaccctgagtacagagaaggctggatgtccgtggggctgtgggatggagctggagggaagggttagctccaaactaaattacatattaaaaagtgatataacttgaggctcaatttttcatcaaattattcaaataatttgttgatttttagctttttttttttttttttggagacggagtttcgctcttgttgcccaggctggagtgcaatggcatgatctcggctcaccgcaacctccgcctcccagattcaagcaattctcctatctcagcctcccaagtagctgggattacaggcatgcaccaccacgcccagctaattttgtatttttagtagagatggggtttctccatgttgaggctggtctcgaactcctgacctcaggtgatctgcccacctcggcctcccaaagtgctgggattacaggcgtaagtcaccgcgcccggccttttttctctttcttttttttttttttgagacagagttttgctcttgttgctcatgctggagtgcaatggcgcaatcttggctcactgcaatctccgcctcccgggttcaagtgattctcctgcctcagcctcctaggtagctgggattacaggcgctcaccaccatgcccggctaaatttttttttttttggattttgagtagaaacggggtttcaccatgttagtctcgaactcctgaccacaggtgatccgcccgctttggcctcccaaagtgctgggattacagatgctcgccactgcgcctggctaatttgttgatttttagaatttgttgtgaggatcctgtgatgtggctatcatcttttgaaagttgtccctgtctttcaaagcgctcctgatacattggagtcattaggtcacttgcagtctgattaaggagagtctttctcttaacgttagtgatattgttccgtgggtggagtcctctctcagcttttgctgaaccagtagcaattacactcacaattttctagcttttctaatacagtgttagatttcatgtagttaagcatctctgttgtcaattaagtaataaacattgttattagaatgtcattaacactaattagaagttgtctagcatggcagctaagagtgtggcttctgttgttgggctggctgtttgaatcctgactcttgacactttttattttgtttgattttatcattttacattgtcttgaactcctggcctcaagcaatcctcccacctcagactcccaaagtgctagcattacaggcgtgagccaccaaacccagcaaacacttacacttaaatgactactctgtatcttaacttcttcatctctacaatggtatgatgattgtaatgatagcactcaaacaagttaataaatgtttacagtggtgcctggtacacagcaaacaccatacagatgctcctcgacttaccgtggggcttcatcctgataaactcatcctaaattgaaaatattgtaagttgaaaatgcacttaatacatacaacccacccaacatcatagcttagcctagcctttttgaaacatgctcagaacacttacattagcccacggttgggcaaaatcacctggcaacacagtaccctgtagaggattcactgtttcccttgtgattttgtggctgactgggagctagtcttgctggcactgtccagtatcgagaatcaagagagtatcttactgcttttttttttttttttcttttttttgagacggagtctggctctgtctcccaggctggagtgcagtggcgcagtctcagctcactgcaacctctgcctcccaggttcaagagattctcctgcctcatcctcccgagtagctgggattacaggtgtgcgccaccacgcccggctaacttttgtatttttagtagagacagggttttgccatgttggccaggctggtcttgaactcctgacctcaggtgatccccccaccttggcctcccaaagtgctggaattacaggcgtgagcaaacgtgcccggccttttactgctttccgatgaatgtatatcaatcgcttttgcgctaccgtaaagtcaaagattgtaagttgaaccatggtaagttgggactgtctgtacaagtgatagttctcactttaggaatgaagctactgttgttgtccatggtgagtgggtattttgggtgagcagaatatgttctattagatggatgtgacattctgtcctcccaggtccctggagcgcctgctgtggtctcagcagccacctgcagaggtcacattagccactccccaacccctgcccttgcctgctcttcccacctctccccaagctccctgagagtcaaagtgccccagaggctgccattcccacaaatggccatgcaaggacagctgcaggggaaggctagcctcaggggcccagagggacacattgggcacttgcccatggggtgccaccaggggtgttgtctctccaggtagaaatatagaaatgggggctggtgtgcagctgctgatgtctctggggtgcgtctggggacctgtgagtgcagggaggtccctggcggggcccgctagggctccttagggttggagggcgcagggcaagggatgaacccaggctggccctccacagtccctatgcctagagggtccctgctgggctgagcattaactttacttgctggactgtgtagagagggtggagtcctggggaggggctaggacaactagggtggtggggggtgcccagcagagcagctttttgccaagtgactcagaaatgtttcagtagtttagccactggcatggctgtggtggtgcatcctggctgaatgctagccctgtccaagggatctgtgtctggaccctcctgagagtccctgtggcacaccagctggggagctctgagctgaggcacagcaaggaaagggactggacagtgtggctggagcagcatgcatgggagaggctgagagagacaggcccactggacccaagcagggaaagaccctggtccagtgcctggcaccttaaaaagcctcccttccacaagatgccccaagagccaggagagggtagtggttaaggtatggacggcctgggtttaagcccaggctcccctgtcctctgaccttgggcaagagagttagtctctccgggtctcagttgccttcactggggaaatggaaacagtaataacagcacttagccaagggtttttgtgaggatttaatgaaacggtgcagtaaagggcttgagagggtttccagccccacagtgatactctgaatacttggtcaatgggaattgtgtacatcgaagcaagaacccatgttacacatttacagtgaaggctttgcaagtggtgctggtgagaatggtgctgcaatgttatcctgagggctactgggacctattttcagagtgggccttataagatcttaaaaggattgcccaggctgcagtgaagaggctgagttggaggagtggaggccaagccgtggaggccaagccaaggaggccagtgaggaggccaatgagccaacagagagaggtccttaggcaggcaagaggcctgagggtccgaggtgggagatacgaaggagtagaaccacctgcaggcagtgtgtgcagttaagaatgtggtcactggtgttggactgcctgggtccagctctgccacttactggctgtgtatcctcgggcaaagaggaggaggtctctgtgcctcagtgttgtcttctgctgtgaaatgagaaaacgatgtgacctacctcttagggttgttacaattaaaaattgtaaatttttaatttacaattttcttggagacagggtctcatgtcatccaggctggaatgcagcagtgagatcatagctcactgcagcctcaaactcctggcttcaagaaatcctcccacctcggccttccaaaattcattataggcaatgactgattatatgcaaagtgtctggaatagggcctggcactattaagtgttagaacacatcctagtgtgattatgttagctagtgtaactattatcagaacttgggtgtgagggaggacctaggatgattctgaggtttgttgctttggtgacatgcatgtcatcaattgggaatttcaagaagaacagatttggctgaaagaaggtgagtcctggggagtctgtgtatatgtgggtaggtaaaggggtctgagtcctggcggaagagaggcctaggttagagaaacaggtggcctgcttatccttggggtgcacctggctgccgaggtcacccatggagagtgggcaggcagggagagaaaaggtcatgccctgaggaacaccaacatttcaggcaactgagaaggagccacctgagggtgggaggaggccagcagagttgggggcatagagagctttgggagggagagtgtcagacgctgctgaggagagtgagatgaagactaacccgaatccataagatttagtaaccgagaagtcttgatgcccttggtgagaaggggcccagtgcagaggggaggacagatgtcagactggttgctttgaggaatgaaagaagacagactggagccaggggatcctaacctccaagggaaatttatttgtctccaccttcccccacctccaggaccaagaaaagcccacttcttgcccaacccatactccagcttggaggcatcggggtcttaaccagagctgaggggggcaagaggaagagaactttgccttcctgagtgcctgctgtgtgctagacctttgtcatgtcacacttgcccagggcggcagtcctgagggcctggtatcagacctcccctcatatcctgaaggacggggctcagagcagttgaggggctgactcaggatggactcctagtccttccctctctgaggagacctaggccatgggaggagcagagaaccacctccagttacccagctgaccaagggcgcggccaagatggtgctaactctcttgccacccatgctggactcctgcctccctaaagtcagctcagcagggggaggactgggtagggaggagaggtgggatgcctgggatgcccctgaaggccagccacccagggctgaacttcacttccataacctccagtctcatgatgtcacatgtggagtcacccccactccagttgtgacccttctgaagagcagcatgaaggggcaggcccttctccacgccaggccctgggctggccactgggggcagaggcagaggagaacatcgtgcccttggagggttttcatgacaacctggagacacaacagatgtttttagtgctaagcatgagtgccggaacatgtaccgagagacatgggcgtgtgtgcagctgtgcataggggagtctggggtgtgatgtggagtgtgtgggagtgggccttagcgggtccatcttggatatctgcctactccatctcatttctgcaggagccagatctggaccccaagccaatcctggagctgcccctggcagagctggcccagcagcttcggaccgaagagctgagtctggagagcatcctctgtagctacttaaagcaggtggtggccagggcacaggatccaagcccggggctctgggctggagtgggggatgtcacttgtcattgttttactcagaggagctgaggggcaggtgtaactctgccactgacttgggaggtggcacatgccacagttacctcagggtggcaggaggggctggggcaaccgagtgccctgctttggtcctggcctcacctggggctgttgtctgctgtcttcactgttgtgcaggcactgaaggtgcaccaggaggtgaactgcctgatggatttcctgggggaatgtgaggaggaactgcaggcattaaagaagcttaagaagagtgagagaggccttctctatggggtccccatgagcctcaaggacacctatgacagcatggtgagcctggggtgtacatgcacacgaatgtgcatatgcacgcttgtgccaccagcctggagcttggtgtgtgacactggggggctcagtgtgtgacaatgggtgagtcatttaaaactgcacagctacgaagcggcaaactgaggtttatacccagaatttgggttccaaaccccaaattctcagccaccacactcttttgccatccgtgaagtgctgcgcttgtgtccccaggggtgtgagagtgtgtgtgaggggggtggaatggggctgaaaatcagccagctggctggttccaccctgacccccatggctggaggcaatgttccttccctgcagggccatgactgtgcatgccgcctggcctagttcctggagaagcctgcgaccaaggacggggtcattatgaaagtgctcaaggcccaaggagccatcccctttgttaagaccaacatcccactgacgctgctcaggtctctgaagcgggctagctggggtcgggggctgggctaagcccagggctgaaacagctctttgaagtcctgattcagggcagagggtgaggagggggctagtcatacagacttcaaagaccagggttcttgggccagccccttctgtccccggggctgagtttctttatcacagaacatgtggatggactccacagtctgtaagggcccttcgggctccaaggttctgtaaagctacactctttttctatcccagtttctctctcaaattgttctatttctacccaggcttctctctttgattgttctccccatcgcttattctctcccttctctactcagcctgtagtgcatctgtgtttcgtgaggaacatgttctcagttctgatggcagagctgtgggctctttggtcctgatattaggagtcatggctggtgtctgatcttggtctttcttgcagcagcagcccctcaccccagctggaagggagcccaggaagcctcagccttagggaggagctcatggagcccaggaagccctggggttgactctggagggtggttggcccccatatggggagaggtctgccgagtgaggctttcaccctcagctcattttcttctgcttcccttagctttgaatgcggcaactcccatctatggccagatgttgagcccactgaacttaaagaagacatgtgggggctcctcagggggtgaggggctctgctggcagaaagggggtccatcctaggcatgggtactgacacaggtgacagcatctgcataccagccagcttctgtggtgtttatggcctctggaccacaggttcccgcctcaggtactcattgatggtggtggtggggtgggctcggacctgcctaagggaactagagggtggggaagtagaggggtctgctcctcccatcaactttcatctacccaactcagtactaggggaagtgggtaggagggcttcaaataactcctgcagtagccatgctaaacataccatatttttccaggtggcagtagaatagaccttccactcattaactcatcagctcattaattcattaatctatacagctatccatccacataccccttctcttactcatcaatctgtccatgtatctatctgtccttcatccattcaatcacccacatggtcatcatctcagtctctatccatcaatcaattttaccattcatccactatttatttaaaagatttctattgactatttactgtgtcagacacaacagctccttgggtactagctacttgggttacttcggtgaacaaaagagacaaatatctcagcccttgaaaaacttacacatactcttccttccaaccatttatccatccatctttccatccatccatttgtgtatccatccatcaatccacatttgtatctctccatccatccatccatccatccatccatccatccatccatccatccatccatccgttcatcgtatatgcatgcatgcatccacccatctctcaacccctctctgtgtacccacaccatggcccctattctggggacatagaccactcttggacccagcccctgcccctgctgtgctcttagacacacaaatgagttagtcagaaagtgatcaggtctgtaagagagggtcaaagcttacaagaggaagctgacattttctttaacagagatttattaaaagcttatactcttgactttcagaggcagggcaagggaagggaaggattcctggaggaggcagcatttgagcgtggttttgagggccagacatgccaagatgatgtggcgtctagaaggctgtaagattgtttgtaagcggctgactttgcctgcagcaatatgcacgtgtggaagggctagaaggggaagccatggagagttagagtcttgaaaagcagtcaaagagatcagactatgctgtgggcagcagagggtcagggaatgttgaagcagctcctatttttgtgggctgcgccctgggggagcacatcgcctgggtgctcaagcctcctagcacccaggcccctcccttcacatgctgagctgggctctgggtcggaatgttttgcagctacactggaattgcctctgccatcaaggggaaaaaaatcgggtaagtcctggtctgtgcctgtggccaccccatttaaagatgaaactgccagtctttctcccaaggacattttgctcagctcatatctccagacagatcagccccacagatgatgactgagagggcagactgcatggttcccacctggcctccccttgtccagtgactcttggccctctgagaagggcttttgtcctgctatctagctttaatctcttccttcgtcctgaccatgaccctggaacccaccctctgaggccaggcagttgggatccccagggcacaacaaatgagaggtgcttgctgggcgcagtggctcatgcctgtaatcccagcactttgggaggctgaggtgggcgatcacttgaggtcaggaattcgagaccagcctggccaacatggtgaaaccccgtctctactagaaatacaaaaattagccaggtgtggtggcgggcacctgtaattccagctactggggaggctgaggcaggagaatcacttgaacccgggaggtggaggttgtagtaagcagagatggtgccactgcactccagcctgggtgacagagaaaaacttcgtctcaaaaaccaacaaacaaaaaacaaaacacaacaagcaaacaaaacgagaggtgcctgcctctctcccctcctctttgtgcagtgaccacggtggctggccccatggcccaggacgtggagagcctggcgctgtgcctgcaagccctgctgagtgaagacatgtaccgactggaccccactgtgctccagatgccctttagggaggaggtaagccaggtgggagagcagacctgggggtttccttgccccccaccatcattcctccctgacctgtctgccatcttaccttcccaggtgaagaccccctttcccaccccaggctgcagtgagtgagaagcccacatgctcagtccagtttgtttccttcccctgctggacaccagctgctttggcttcttggctatctggagccatagcttgtaagtgcccccaaagagggcctccagtgccatatacccaacccatgcagttagaatactcagcaagtgtggttgagagggtgtggcatccagttaagctgggtttttaaccctctaggtaaccctggccaagtcacatctcttctttcagccttagcctccccatcaatacaataaagaggttaggctgggagattactccacacccttctgtctacagcagccttcatttattcgttaattcattcaacaacatttgcttgtaccagttgtgtgccaggctctgcgtgtctcatcctaacactctatagagtgagcagtgctcctcccatttacagctggggagactgaggggaagtgaaatgacttgcctaagatcatgtagttagtaactggcagagctggctttgaacccagccctatctaactgcagaaccctctccatagggcagtttctgtctacgtcccggcaatgtctgttcctcggattccctacacccctcctagcattatcaacctgagatcattgtatatcatccatgatttgcccctacaaacatgtgttgtgtgacgggtgaggggcggctgcctttctggcagcaccccacttcccaggactaggggccctccatctcagaccctggtctgggtatttgtccctatagatctccagcctcatattctcctaacatttctttagcttaaagatatttgagtctatgcatgacttactcacctgcccacccactcaactccaaccatccattcacccactcacccacatatgcattcaaccctctgcccacccaactacccaccatctcatacatacatccacccacccacccaggagtctgtctaccatctatctactatccaccccatctgcccaaccacccatctcatccatttctctttcctccaggggtttccgcagagcacctagagcctggagagtatatagggaggctcccagggggtcttggggtgtccacatggattcccccctttgtgaggacagctgtagaccaaggccctgcccttaaagtctggctcctggatagagtggggccaccttgtccccagcacaatctctcctccgagctccatccagccccttgtgcccctaggtttacaccagtaaccggccccttcgaattggctactatgaatcagatggttacatccagccatcccctagcatggccagggctgtgcagctcacctcctggctgctccaggatgcttgacaccaggtagtctcacctggtcctgggtgagagagagtctgggccagtgcgaggatgctgggcggggccatccttggagacaaaggtggctacatctgcgtttgaggtgctgagataactgtgttccccctatgcttcctggagaagactgatgggatggaggtggggatagggtgagccctaccctagaaggaaggcattaagcttttgtgcttcctccttcggtggtggagattcagggactcactcctataattccttcagcttgggtctctgttgcctccatcaagtggccgtaaggagctttctgtctccaaaatccctaccttagccctaccccaaactcccctgcccccagtggcttgtcctggcctcacttcccctttgagattctaccatgtgatcttgggctagccttttaacctctctgggcttgttttctacccaatgcggtggctgtgaagattaaatgtggttccatagataaagcacttggcacgctggctggatcacagtgaagcatgaaggaaatgagggctgctctcgttctgttctgtcacatctgtgtgtgagggtgagggagtggggtggcaggagagcaaccagtgacacaggcctcccatgccatgctgaggcgctgaggtggacggagatgcacgagatgatgtggcatccttcttgaaatcttgggggatgcagagacagagaaccaggcagggtcggggaagctccagacactgactctgcctctgcctccccaggttatccccttctccatcccccaggcagaatacgccatcaaagacttgtacacggggggatgtttactgatggaggggccactcttctagagaagctatacgttatctgctgggactcaggggtggggcatggtggaaacaaggtaggggagtgggctggagccaacctgagtcccaggagggaaactgggggcctgggctggggtgcctctgcctaatagtgtgaccttatgccgcaaaccacacactgggcctgtctttaggatgcacctgttccgggggtggggcagaagtacatctttgggtttggcctccttcttgtctacggcgtggaagttgggtggctgtgggggcaggccactggctaagggctgtgacttacccatctgcgactggttcctcagagagggggacattgtggatcccagcataaagggcatggtcaaccagctctgcctgccagaccccttcaaatgtttcttggcctggatcccaaagtacatagtaagtgcaggccctagtcagggagggctttggaagggcagggagcacagggagtaggaggggctcagaaagcagagggagctcacagaaggagtggaagtggggtcagagaggaggatgaggcccagagaatggtggtagctcagagaggggttcaaaatggggaagaagaatgaagggctgggtgcacagtggctcatgtatgtaatcccagcactttgggaggccaaggtaggaagatcacttgagcccaggagtctgagaccagcctgggcaacatagtgagactccattctctaaaaagaatggaaaaaaaaatagctgggcatggtggtgcatgcctgtggtcccagctactcaggaggctgaggtgggagtatcacttgagcccagaagatcaaggctgcagtgagctgagattatgcactgcactccagcttgggtgacaagtaagactctgactcaaaaaaaataaaaaaaaattaattaaaacaaataatgaaagaaggggatggggctaaaagagtagggtgctcacagagaggggagggggtttcagagaggaggctcagaaagggggaagggcatttggagggctacagggccagtgtgagctcagggcttggtgaagtggtgtaggcttgttgaggatcggagggttccacgtcagtgcgttgagcaatgctacccttcttggaccccctcctgggcaggctgactgtttccctgtgggttctgaagttggactccccctctcagcccccctctaggatccccaaactagccagcatcttgaagagattcgtggagtggggtgagtctccctagggccagctcttgctccaatggttgtccatgggatggtgggaattgaggaggggcatgaggctagagctggtatccactaaggggggatctatttagatttcggactctaattagggttttaggatcatgcctgacattagcttagattgagacttttgattggtgttgggactttatttggagttaagatctgaattaaggccgggtgtggtggctcatgcctgtaatcccagcactttgggaggctgagcggggaggatcacttgaggccaggggttcaagaccagccaggacaacatgatgaaaccctgtccctactaaaaatacaaaaatcagcgggtgtggtggtatgtgtctttatcccagctactcgggaggctgaggcacgagaatcacttgaacccaggaggtggagcttgcagtgggccaagatggtgccactgcactctagcctgggtgatagagatagactctgtctcaagggaaaaaaaaatctgaattaaggctaggttgaggtaaaatttgggactgaagttgagattaggttttatttggggatgggcttaagactgaggctggggttggagttggtttgagttggggttggtggggcgaagatagatttggaagagggttgggactgaggctggagttggggtggggctagagttagggttagagatgaggttgggagaggctggtatgggcttgggtttgctgttgggcttggcctggtggggttggcatgaagatgctgggcagaattgggctggagtggactgagggctaactgggtgcctcacagattagggtaaggagcctgtggcctttgaggcagcccatgagttcctgtgactggtggaatggggggtagattgaccagaggatgtgtgctcttggggaccttgagcaggcaagatgtcttggccaggggacaagacacggggtcactcccagcccatcagctgatttgcagcgtgcactgaggccttggttgtcatgtccccatttgtataaaagggttccctcccatgctgacctttgaacttgtcagagtcttcctcattctttcaggacacccaagaaactgtgggaacagcacacagcagtggaggtaatgcctgtctgggaagaccttgaggggctgctggagctggggctgcagacacctgggtagtgccctgagtggtcagagttatgaactggcctgcagagaaggcccagctggacctgggtgggggggcttggtgacctcagaagttattctagtccatctccctagagcattgtccccaaatccttgtgacctgaaattcagcttcccatcccttcacctctgtccctgggaagatcctgaacctccacaggtatctcaggctgaagcttatagcctgagacttcctcctggtgtgcaactcagtgctgcctggcagcatctgaccttgtctggcaaacagtaacccctgccttcctacccctcccatccctcactgtccctgcaggaatatgagcaagagttcatagccaagtggaggtccctggacctggatgtgctgctggtgccagttctgggctctgccttctatataggctcttcctccctagcatcaggtgagagcacactgggtcttggtggggttgagattgggagtccgggactcctgagtcctgccccagcttctgtgatcttgccctctatctccattaactttttaaaaatatttcttaaattgagataaaagtcagataacacaaacttaccattttaaagtgtacaattaagtggtttttaatatttcaaaatgtcgtgcaaccaccaccattatctaatgtctgaacatttctgttaccctgaaaggaaaacttgtacctgttagcaatttccattcactttaaaaatgaactttatggaagtataatttacatgcaataaaattcaccgattttaagtataatttgatgaattttgacaaatgtatactgttgtataaccaccactataatcagaaatacagaacagaatatatttttagattttacagatacatgttccatcacccccaaatttccctcatgtctctgcagttcactctatccctaaccccagtaaccactgatctgctttctgtcaccatagttttgccttttctagaatttcatacaaatggaatcaaagggtatgaagcttttgtgtttggcttcttccacctagcacatccatttactgtttttttttttttttttttttttttttttttttttttgagacagagtcttgctctgtcacccaggctggagcgcagtggcatgatctcagctcactgcaacctcctctgcctcctgatttcaagcaattctcctgcctcagcctcccaagtagctggaattacaggtgtgtgccaccacgtccagctaatctttgcatttttagtagagacggggttgcgccatgttggctaggctggtctcaaactcctaacctcaggtgatccacccacctcagcctcccaaagtcctggcattacaggcgtgagccactgtgcccagcccatccatttactcttaacatgccctctgctgccctacttcaaaaggggtcttcagcccagcctgtccaaaacatgggctcaggacagggtaatatctgggccatccctgggtcccatgcacaggtactggtctcaaaggtgctacccaaggcaggataaaactcagttccaaacctgagcctggactcctctcccctgaccttaagaacatgtcctcctgggtcccccgactgtggccagccaaaggctcatcccacgcctgactctccctgcacacatgtggctgctgcagaagagctgtcctttcaactccaggtggcgctgtacacccttactatcttgaagtccggtacacaggagggcgtgggctgaatcctctgccatccactagctgtgtagccttagaaaaggctaatcctgcccctaatcctgccacctcgatttcctcacttgtacacagtcaatagtaatccacacctcacagagtggagaggattcaagggatcagcaatgtgatgaggccagcacagtgcctggcactgagtgaggcttctgcaatgcagattccgtccttccctccaccctggggagagcatgaggccattgtcaagatgacccctgacacaaattggctagtccgagcccagagcgctgaagttcccagaaggaccgggagggggcgcccacccacattcttccccacctgagtctgcgctgacgatttcctgggcttatctggatcttcctgcagaaagtcagtcttatgtgaccctgtacaacctcctggactttcccgcgggcgtggtgcctgtcactatcgtgacactacaggacgaggaggaactggccttctacaaggggtgctacggagatagttctgacaaaaatttctcagaggtcagtttccttctccgagcctctcccggagcggggacaaaccagggctggttctctccgggttggggcccctgacggtagtggtggagagagtagggcgggactggtcattcctggtgttcaccctttggcacttatgctagtttcaccccaaccctgaggacacatcatttgacctccttgtcagccccatccatgtcaggggagaaaactttgcaaaaccagtggttttctttgtatttcttctgcctcctcctcctccccctccccctccccctcttcctccttctcctcctcctcttcctcctcctcctccttctccccctccttcttctttttcttcttctcctcctcctcctcctcctcctcctccttctccccctccttctccttctccttcttcctccttttccttctccttctccttctccttcttcctccttttccttctccttctccttcttttttgagacagagtcttgctctatcgcccaggctggagtgcagtggcacgatctcggctcactgcaacctctgcctcctgggttcaagtgattctcctgcctcagcctcccaagtagctgggattacaggcacctgccaccacgcccggctaatttttttttttttttttgagatggaatctcactcttttgcccaggctgatgtgcagtggtgcaatctcagctcactgcaacctccacatcctgagtttgagccatcctcctgcctctcagcctcccaagtagctgggactacaggcatgcaccaccatgctcggctaatttttgtaattttagtagagacacggtttcaccatgttggtcaggctggtctcaaactcctggcctcaagtgatctgcctgcctcggcctcccaatgtgctgggattacaggtgtgagccattgcgcccggccttctttgcattgctgtaggtaaaaatgatctcagaggcagggagggcagagcagggcaaaagccgctggttatgagcttactgtgtatctgctctggatatgacctctcttgggacctctgtttcttcaccaggaaaatgggaataaaaacatctactttgtagggttgtgctaaaggttaattaatttgaaaaagtgaatgaagcaatttgcataaggtcttgtgtgtaggaagtgttcgataaatactatgattagtaagtcagagtggtttcataaaagaaaatattaccaaatatttaactgcagggtctaaaataacacacctgactttggtgagagagagaaggagagagaggaagagaaagaggccgactctgaaacatatgcacgtatctgagtcagacattaagtaacttactttttctggaaattgattttagtgctagagttacccagtggaactgctgacctgaattctgagaaaataacaataatgacactatctcatgtgtcttgagcacttactctgttccaggagctgtttaaaagtgccgtgtataaatattaaatcattaaattcaataactctcctgtgaggttttttaaatgaggaaaatggaggcacagacagattaagggactgggccaaagccacacagccaattgaagtggaggagctaggacttgaaacaggtgatctgactccagagacaaaggcaaataaagcctcaaatgatatcatcacaaagcaaagaaaacaggtttgaattcctacaaggacgtttggatttcgtggcagggactcaggcttagcccccatgttcctgggcctgttttgggccaaggcaatgctttcactgtggaagggtaaccaggctctggatcagggattagcatgctcttctttctcttgcttgaacattgagtggatgctcggctttctctttcgtcattataatcagcattctgcacagggagcaagttttacatgttaaccctgaagaactatgggcaataaaatcagaacagtcttttcaggtttcactgagagctgaggaagcctggaattctgagatctaggtcatttttaccttaatatagattgggaaagggatgtttggactaaagcatacctagaccaaccgttggtacggaggcccagaatagcatgggtgatgaacagagccaggcaaggggcctgtgaagcaggctctgagttcccgaccttctctactggcaggcggtaagaggatccgtcggagttctggtgactgtgcagtgcattgctttgccatgggaagaggagctgtgtctccggttcatgaaggaggtggacaccttggtcaagaatcagagggggcccaagtgataggctcctggaatggagtaacagctcatgaaacacggggctggttgtggtggctcatacttgtaatcccagcagttcaggaggcagaggctggcagatcgcttgaggccacgagtttgagaccaacctgggcaacatagtgagaccctgcttctaaagcattttcttggtgttactcctgtagatcctcacccaagtgtgctcctgatgccccttccttctcatgaataccatgtccaccttatgtctcctccttctggaaccccaccaggttccttttctttgttggtccctctgtgtgggtgctcaatattcctcagatgggcccaggatggggagcagggtgaggagctcaataaacattttctgactggc

SEQ ID NO: 6 - DNA, 18829 bp, Homo sapiens
tttcgctcttgttgcccaggctggagtgcaatggcatgatctcggctcaccgcaacctccgcctcccagattcaagcaattctcctatctcagcctcccaagtagctgggattacaggcatgcaccaccacgcccagctaattttgtatttttagtagagatggggtttctccatgttgaggctggtctcgaactcctgacctcaggtgatctgcccacctcggcctcccaaagtgctgggattacaggcgtaagtcaccgcgcccggccttttttctctttcttttttttttttttgagacagagttttgctcttgttgctcatgctggagtgcaatggcgcaatcttggctcactgcaatctccgcctcccgggttcaagtgattctcctgcctcagcctcctaggtagctgggattacaggcgctcaccaccatgcccggctaaatttttttttttttggattttgagtagaaacggggtttcaccatgttagtctcgaactcctgaccacaggtgatccgcccgctttggcctcccaaagtgctgggattacagatgctcgccactgcgcctggctaatttgttgatttttagaatttgttgtgaggatcctgtgatgtggctatcatcttttgaaagttgtccctgtctttcaaagcgctcctgatacattggagtcattaggtcacttgcagtctgattaaggagagtctttctcttaacgttagtgatattgttccgtgggtggagtcctctctcagcttttgctgaaccagtagcaattacactcacaattttctagcttttctaatacagtgttagatttcatgtagttaagcatctctgttgtcaattaagtaataaacattgttattagaatgtcattaacactaattagaagttgtctagcatggcagctaagagtgtggcttctgttgttgggctggctgtttgaatcctgactcttgacactttttattttgtttgattttatcattttacattgtcttgaactcctggcctcaagcaatcctcccacctcagactcccaaagtgctagcattacaggcgtgagccaccaaacccagcaaacacttacacttaaatgactactctgtatcttaacttcttcatctctacaatggtatgatgattgtaatgatagcactcaaacaagttaataaatgtttacagtggtgcctggtacacagcaaacaccatacagatgctcctcgacttaccgtggggcttcatcctgataaactcatcctaaattgaaaatattgtaagttgaaaatgcacttaatacatacaacccacccaacatcatagcttagcctagcctttttgaaacatgctcagaacacttacattagcccacggttgggcaaaatcacctggcaacacagtaccctgtagaggattcactgtttcccttgtgattttgtggctgactgggagctagtcttgctggcactgtccagtatcgagaatcaagagagtatcttactgcttttttttttttttttcttttttttgagacggagtctggctctgtctcccaggctggagtgcagtggcgcagtctcagctcactgcaacctctgcctcccaggttcaagagattctcctgcctcatcctcccgagtagctgggattacaggtgtgcgccaccacgcccggctaacttttgtatttttagtagagacagggttttgccatgttggccaggctggtcttgaactcctgacctcaggtgatccccccaccttggcctcccaaagtgctggaattacaggcgtgagcaaacgtgcccggccttttactgctttccgatgaatgtatatcaatcgcttttgcgctaccgtaaagtcaaagattgtaagttgaaccatggtaagttgggactgtctgtacaagtgatagttctcactttaggaatgaagctactgttgttgtccatggtgagtgggtattttgggtgagcagaatatgttctattagatggatgtgacattctgtcctcccaggtccctggagcgcctgctgtggtctcagcagccacctgcagaggtcacattagccactccccaacccctgcccttgcctgctcttcccacctctccccaagctccctgagagtcaaagtgccccagaggctgccattcccacaaatggccatgcaaggacagctgcaggggaaggctagcctcaggggcccagagggacacattgggcacttgcccatggggtgccaccaggggtgttgtctctccaggtagaaatatagaaatgggggctggtgtgcagctgctgatgtctctggggtgcgtctggggacctgtgagtgcagggaggtccctggcggggcccgctagggctccttagggttggagggcgcagggcaagggatgaacccaggctggccctccacagtccctatgcctagagggtccctgctgggctgagcattaactttacttgctggactgtgtagagagggtggagtcctggggaggggctaggacaactagggtggtggggggtgcccagcagagcagctttttgccaagtgactcagaaatgtttcagtagtttagccactggcatggctgtggtggtgcatcctggctgaatgctagccctgtccaagggatctgtgtctggaccctcctgagagtccctgtggcacaccagctggggagctctgagctgaggcacagcaaggaaagggactggacagtgtggctggagcagcatgcatgggagaggctgagagagacaggcccactggacccaagcagggaaagaccctggtccagtgcctggcaccttaaaaagcctcccttccacaagatgccccaagagccaggagagggtagtggttaaggtatggacggcctgggtttaagcccaggctcccctgtcctctgaccttgggcaagagagttagtctctccgggtctcagttgccttcactggggaaatggaaacagtaataacagcacttagccaagggtttttgtgaggatttaatgaaacggtgcagtaaagggcttgagagggtttccagccccacagtgatactctgaatacttggtcaatgggaattgtgtacatcgaagcaagaacccatgttacacatttacagtgaaggctttgcaagtggtgctggtgagaatggtgctgcaatgttatcctgagggctactgggacctattttcagagtgggccttataagatcttaaaaggattgcccaggctgcagtgaagaggctgagttggaggagtggaggccaagccgtggaggccaagccaaggaggccagtgaggaggccaatgagccaacagagagaggtccttaggcaggcaagaggcctgagggtccgaggtgggagatacgaaggagtagaaccacctgcaggcagtgtgtgcagttaagaatgtggtcactggtgttggactgcctgggtccagctctgccacttactggctgtgtatcctcgggcaaagaggaggaggtctctgtgcctcagtgttgtcttctgctgtgaaatgagaaaacgatgtgacctacctcttagggttgttacaattaaaaattgtaaatttttaatttacaattttcttggagacagggtctcatgtcatccaggctggaatgcagcagtgagatcatagctcactgcagcctcaaactcctggcttcaagaaatcctcccacctcggccttccaaaattcattataggcaatgactgattatatgcaaagtgtctggaatagggcctggcactattaagtgttagaacacatcctagtgtgattatgttagctagtgtaactattatcagaacttgggtgtgagggaggacctaggatgattctgaggtttgttgctttggtgacatgcatgtcatcaattgggaatttcaagaagaacagatttggctgaaagaaggtgagtcctggggagtctgtgtatatgtgggtaggtaaaggggtctgagtcctggcggaagagaggcctaggttagagaaacaggtggcctgcttatccttggggtgcacctggctgccgaggtcacccatggagagtgggcaggcagggagagaaaaggtcatgccctgaggaacaccaacatttcaggcaactgagaaggagccacctgagggtgggaggaggccagcagagttgggggcatagagagctttgggagggagagtgtcagacgctgctgaggagagtgagatgaagactaacccgaatccataagatttagtaaccgagaagtcttgatgcccttggtgagaaggggcccagtgcagaggggaggacagatgtcagactggttgctttgaggaatgaaagaagacagactggagccaggggatcctaacctccaagggaaatttatttgtctccaccttcccccacctccaggaccaagaaaagcccacttcttgcccaacccatactccagcttggaggcatcggggtcttaaccagagctgaggggggcaagaggaagagaactttgccttcctgagtgcctgctgtgtgctagacctttgtcatgtcacacttgcccagggcggcagtcctgagggcctggtatcagacctcccctcatatcctgaaggacggggctcagagcagttgaggggctgactcaggatggactcctagtccttccctctctgaggagacctaggccatgggaggagcagagaaccacctccagttacccagctgaccaagggcgcggccaagatggtgctaactctcttgccacccatgctggactcctgcctccctaaagtcagctcagcagggggaggactgggtagggaggagaggtgggatgcctgggatgcccctgaaggccagccacccagggctgaacttcacttccataacctccagtctcatgatgtcacatgtggagtcacccccactccagttgtgacccttctgaagagcagcatgaaggggcaggcccttctccacgccaggccctgggctggccactgggggcagaggcagaggagaacatcgtgcccttggagggttttcatgacaacctggagacacaacagatgtttttagtgctaagcatgagtgccggaacatgtaccgagagacatgggcgtgtgtgcagctgtgcataggggagtctggggtgtgatgtggagtgtgtgggagtgggccttagcgggtccatcttggatatctgcctactccatctcatttctgcaggagccagatctggaccccaagccaatcctggagctgcccctggcagagctggcccagcagcttcggaccgaagagctgagtctggagagcatcctctgtagctacttaaagcaggtggtggccagggcacaggatccaagcccggggctctgggctggagtgggggatgtcacttgtcattgttttactcagaggagctgaggggcaggtgtaactctgccactgacttgggaggtggcacatgccacagttacctcagggtggcaggaggggctggggcaaccgagtgccctgctttggtcctggcctcacctggggctgttgtctgctgtcttcactgttgtgcaggcactgaaggtgcaccaggaggtgaactgcctgatggatttcctgggggaatgtgaggaggaactgcaggcattaaagaagcttaagaagagtgagagaggccttctctatggggtccccatgagcctcaaggacacctatgacagcatggtgagcctggggtgtacatgcacacgaatgtgcatatgcacgcttgtgccaccagcctggagcttggtgtgtgacactggggggctcagtgtgtgacaatgggtgagtcatttaaaactgcacagctacgaagcggcaaactgaggtttatacccagaatttgggttccaaaccccaaattctcagccaccacactcttttgccatccgtgaagtgctgcgcttgtgtccccaggggtgtgagagtgtgtgtgaggggggtggaatggggctgaaaatcagccagctggctggttccaccctgacccccatggctggaggcaatgttccttccctgcagggccatgactgtgcatgccgcctggcctagttcctggagaagcctgcgaccaaggacggggtcattatgaaagtgctcaaggcccaaggagccatcccctttgttaagaccaacatcccactgacgctgctcaggtctctgaagcgggctagctggggtcgggggctgggctaagcccagggctgaaacagctctttgaagtcctgattcagggcagagggtgaggagggggctagtcatacagacttcaaagaccagggttcttgggccagccccttctgtccccggggctgagtttctttatcacagaacatgtggatggactccacagtctgtaagggcccttcgggctccaaggttctgtaaagctacactctttttctatcccagtttctctctcaaattgttctatttctacccaggcttctctctttgattgttctccccatcgcttattctctcccttctctactcagcctgtagtgcatctgtgtttcgtgaggaacatgttctcagttctgatggcagagctgtgggctctttggtcctgatattaggagtcatggctggtgtctgatcttggtctttcttgcagcagcagcccctcaccccagctggaagggagcccaggaagcctcagccttagggaggagctcatggagcccaggaagccctggggttgactctggagggtggttggcccccatatggggagaggtctgccgagtgaggctttcaccctcagctcattttcttctgcttcccttagctttgaatgcggcaactcccatctatggccagatgttgagcccactgaacttaaagaagacatgtgggggctcctcagggggtgaggggctctgctggcagaaagggggtccatcctaggcatgggtactgacacaggtgacagcatctgcataccagccagcttctgtggtgtttatggcctctggaccacaggttcccgcctcaggtactcattgatggtggtggtggggtgggctcggacctgcctaagggaactagagggtggggaagtagaggggtctgctcctcccatcaactttcatctacccaactcagtactaggggaagtgggtaggagggcttcaaataactcctgcagtagccatgctaaacataccatatttttccaggtggcagtagaatagaccttccactcattaactcatcagctcattaattcattaatctatacagctatccatccacataccccttctcttactcatcaatctgtccatgtatctatctgtccttcatccattcaatcacccacatggtcatcatctcagtctctatccatcaatcaattttaccattcatccactatttatttaaaagatttctattgactatttactgtgtcagacacaacagctccttgggtactagctacttgggttacttcggtgaacaaaagagacaaatatctcagcccttgaaaaacttacacatactcttccttccaaccatttatccatccatctttccatccatccatttgtgtatccatccatcaatccacatttgtatctctccatccatccatccatccatccatccatccatccatccatccatccatccatccgttcatcgtatatgcatgcatgcatccacccatctctcaacccctctctgtgtacccacaccatggcccctattctggggacatagaccactcttggacccagcccctgcccctgctgtgctcttagacacacaaatgagttagtcagaaagtgatcaggtctgtaagagagggtcaaagcttacaagaggaagctgacattttctttaacagagatttattaaaagcttatactcttgactttcagaggcagggcaagggaagggaaggattcctggaggaggcagcatttgagcgtggttttgagggccagacatgccaagatgatgtggcgtctagaaggctgtaagattgtttgtaagcggctgactttgcctgcagcaatatgcacgtgtggaagggctagaaggggaagccatggagagttagagtcttgaaaagcagtcaaagagatcagactatgctgtgggcagcagagggtcagggaatgttgaagcagctcctatttttgtgggctgcgccctgggggagcacatcgcctgggtgctcaagcctcctagcacccaggcccctcccttcacatgctgagctgggctctgggtcggaatgttttgcagctacactggaattgcctctgccatcaaggggaaaaaaatcgggtaagtcctggtctgtgcctgtggccaccccatttaaagatgaaactgccagtctttctcccaaggacattttgctcagctcatatctccagacagatcagccccacagatgatgactgagagggcagactgcatggttcccacctggcctccccttgtccagtgactcttggccctctgagaagggcttttgtcctgctatctagctttaatctcttccttcgtcctgaccatgaccctggaacccaccctctgaggccaggcagttgggatccccagggcacaacaaatgagaggtgcttgctgggcgcagtggctcatgcctgtaatcccagcactttgggaggctgaggtgggcgatcacttgaggtcaggaattcgagaccagcctggccaacatggtgaaaccccgtctctactagaaatacaaaaattagccaggtgtggtggcgggcacctgtaattccagctactggggaggctgaggcaggagaatcacttgaacccgggaggtggaggttgtagtaagcagagatggtgccactgcactccagcctgggtgacagagaaaaacttcgtctcaaaaaccaacaaacaaaaaacaaaacacaacaagcaaacaaaacgagaggtgcctgcctctctcccctcctctttgtgcagtgaccacggtggctggccccatggcccaggacgtggagagcctggcgctgtgcctgcaagccctgctgagtgaagacatgtaccgactggaccccactgtgctccagatgccctttagggaggaggtaagccaggtgggagagcagacctgggggtttccttgccccccaccatcattcctccctgacctgtctgccatcttaccttcccaggtgaagaccccctttcccaccccaggctgcagtgagtgagaagcccacatgctcagtccagtttgtttccttcccctgctggacaccagctgctttggcttcttggctatctggagccatagcttgtaagtgcccccaaagagggcctccagtgccatatacccaacccatgcagttagaatactcagcaagtgtggttgagagggtgtggcatccagttaagctgggtttttaaccctctaggtaaccctggccaagtcacatctcttctttcagccttagcctccccatcaatacaataaagaggttaggctgggagattactccacacccttctgtctacagcagccttcatttattcgttaattcattcaacaacatttgcttgtaccagttgtgtgccaggctctgcgtgtctcatcctaacactctatagagtgagcagtgctcctcccatttacagctggggagactgaggggaagtgaaatgacttgcctaagatcatgtagttagtaactggcagagctggctttgaacccagccctatctaactgcagaaccctctccatagggcagtttctgtctacgtcccggcaatgtctgttcctcggattccctacacccctcctagcattatcaacctgagatcattgtatatcatccatgatttgcccctacaaacatgtgttgtgtgacgggtgaggggcggctgcctttctggcagcaccccacttcccaggactaggggccctccatctcagaccctggtctgggtatttgtccctatagatctccagcctcatattctcctaacatttctttagcttaaagatatttgagtctatgcatgacttactcacctgcccacccactcaactccaaccatccattcacccactcacccacatatgcattcaaccctctgcccacccaactacccaccatctcatacatacatccacccacccacccaggagtctgtctaccatctatctactatccaccccatctgcccaaccacccatctcatccatttctctttcctccaggggtttccgcagagcacctagagcctggagagtatatagggaggctcccagggggtcttggggtgtccacatggattcccccctttgtgaggacagctgtagaccaaggccctgcccttaaagtctggctcctggatagagtggggccaccttgtccccagcacaatctctcctccgagctccatccagccccttgtgcccctaggtttacaccagtaaccggccccttcgaattggctactatgaatcagatggttacatccagccatcccctagcatggccagggctgtgcagctcacctcctggctgctccaggatgcttgacaccaggtagtctcacctggtcctgggtgagagagagtctgggccagtgcgaggatgctgggcggggccatccttggagacaaaggtggctacatctgcgtttgaggtgctgagataactgtgttccccctatgcttcctggagaagactgatgggatggaggtggggatagggtgagccctaccctagaaggaaggcattaagcttttgtgcttcctccttcggtggtggagattcagggactcactcctataattccttcagcttgggtctctgttgcctccatcaagtggccgtaaggagctttctgtctccaaaatccctaccttagccctaccccaaactcccctgcccccagtggcttgtcctggcctcacttcccctttgagattctaccatgtgatcttgggctagccttttaacctctctgggcttgttttctacccaatgcggtggctgtgaagattaaatgtggttccatagataaagcacttggcacgctggctggatcacagtgaagcatgaaggaaatgagggctgctctcgttctgttctgtcacatctgtgtgtgagggtgagggagtggggtggcaggagagcaaccagtgacacaggcctcccatgccatgctgaggcgctgaggtggacggagatgcacgagatgatgtggcatccttcttgaaatcttgggggatgcagagacagagaaccaggcagggtcggggaagctccagacactgactctgcctctgcctccccaggttatccccttctccatcccccaggcagaatacgccatcaaagacttgtacacggggggatgtttactgatggaggggccactcttctagagaagctatacgttatctgctgggactcaggggtggggcatggtggaaacaaggtaggggagtgggctggagccaacctgagtcccaggagggaaactgggggcctgggctggggtgcctctgcctaatagtgtgaccttatgccgcaaaccacacactgggcctgtctttaggatgcacctgttccgggggtggggcagaagtacatctttgggtttggcctccttcttgtctacggcgtggaagttgggtggctgtgggggcaggccactggctaagggctgtgacttacccatctgcgactggttcctcagagagggggacattgtggatcccagcataaagggcatggtcaaccagctctgcctgccagaccccttcaaatgtttcttggcctggatcccaaagtacatagtaagtgcaggccctagtcagggagggctttggaagggcagggagcacagggagtaggaggggctcagaaagcagagggagctcacagaaggagtggaagtggggtcagagaggaggatgaggcccagagaatggtggtagctcagagaggggttcaaaatggggaagaagaatgaagggctgggtgcacagtggctcatgtatgtaatcccagcactttgggaggccaaggtaggaagatcacttgagcccaggagtctgagaccagcctgggcaacatagtgagactccattctctaaaaagaatggaaaaaaaaatagctgggcatggtggtgcatgcctgtggtcccagctactcaggaggctgaggtgggagtatcacttgagcccagaagatcaaggctgcagtgagctgagattatgcactgcactccagcttgggtgacaagtaagactctgactcaaaaaaaataaaaaaaaattaattaaaacaaataatgaaagaaggggatggggctaaaagagtagggtgctcacagagaggggagggggtttcagagaggaggctcagaaagggggaagggcatttggagggctacagggccagtgtgagctcagggcttggtgaagtggtgtaggcttgttgaggatcggagggttccacgtcagtgcgttgagcaatgctacccttcttggaccccctcctgggcaggctgactgtttccctgtgggttctgaagttggactccccctctcagcccccctctaggatccccaaactagccagcatcttgaagagattcgtggagtggggtgagtctccctagggccagctcttgctccaatggttgtccatgggatggtgggaattgaggaggggcatgaggctagagctggtatccactaaggggggatctatttagatttcggactctaattagggttttaggatcatgcctgacattagcttagattgagacttttgattggtgttgggactttatttggagttaagatctgaattaaggccgggtgtggtggctcatgcctgtaatcccagcactttgggaggctgagcggggaggatcacttgaggccaggggttcaagaccagccaggacaacatgatgaaaccctgtccctactaaaaatacaaaaatcagcgggtgtggtggtatgtgtctttatcccagctactcgggaggctgaggcacgagaatcacttgaacccaggaggtggagcttgcagtgggccaagatggtgccactgcactctagcctgggtgatagagatagactctgtctcaagggaaaaaaaaatctgaattaaggctaggttgaggtaaaatttgggactgaagttgagattaggttttatttggggatgggcttaagactgaggctggggttggagttggtttgagttggggttggtggggcgaagatagatttggaagagggttgggactgaggctggagttggggtggggctagagttagggttagagatgaggttgggagaggctggtatgggcttgggtttgctgttgggcttggcctggtggggttggcatgaagatgctgggcagaattgggctggagtggactgagggctaactgggtgcctcacagattagggtaaggagcctgtggcctttgaggcagcccatgagttcctgtgactggtggaatggggggtagattgaccagaggatgtgtgctcttggggaccttgagcaggcaagatgtcttggccaggggacaagacacggggtcactcccagcccatcagctgatttgcagcgtgcactgaggccttggttgtcatgtccccatttgtataaaagggttccctcccatgctgacctttgaacttgtcagagtcttcctcattctttcaggacacccaagaaactgtgggaacagcacacagcagtggaggtaatgcctgtctgggaagaccttgaggggctgctggagctggggctgcagacacctgggtagtgccctgagtggtcagagttatgaactggcctgcagagaaggcccagctggacctgggtgggggggcttggtgacctcagaagttattctagtccatctccctagagcattgtccccaaatccttgtgacctgaaattcagcttcccatcccttcacctctgtccctgggaagatcctgaacctccacaggtatctcaggctgaagcttatagcctgagacttcctcctggtgtgcaactcagtgctgcctggcagcatctgaccttgtctggcaaacagtaacccctgccttcctacccctcccatccctcactgtccctgcaggaatatgagcaagagttcatagccaagtggaggtccctggacctggatgtgctgctggtgccagttctgggctctgccttctatataggctcttcctccctagcatcaggtgagagcacactgggtcttggtggggttgagattgggagtccgggactcctgagtcctgccccagcttctgtgatcttgccctctatctccattaactttttaaaaatatttcttaaattgagataaaagtcagataacacaaacttaccattttaaagtgtacaattaagtggtttttaatatttcaaaatgtcgtgcaaccaccaccattatctaatgtctgaacatttctgttaccctgaaaggaaaacttgtacctgttagcaatttccattcactttaaaaatgaactttatggaagtataatttacatgcaataaaattcaccgattttaagtataatttgatgaattttgacaaatgtatactgttgtataaccaccactataatcagaaatacagaacagaatatatttttagattttacagatacatgttccatcacccccaaatttccctcatgtctctgcagttcactctatccctaaccccagtaaccactgatctgctttctgtcaccatagttttgccttttctagaatttcatacaaatggaatcaaagggtatgaagcttttgtgtttggcttcttccacctagcacatccatttactgtttttttttttttttttttttttttttttttttttttgagacagagtcttgctctgtcacccaggctggagcgcagtggcatgatctcagctcactgcaacctcctctgcctcctgatttcaagcaattctcctgcctcagcctcccaagtagctggaattacaggtgtgtgccaccacgtccagctaatctttgcatttttagtagagacggggttgcgccatgttggctaggctggtctcaaactcctaacctcaggtgatccacccacctcagcctcccaaagtcctggcattacaggcgtgagccactgtgcccagcccatccatttactcttaacatgccctctgctgccctacttcaaaaggggtcttcagcccagcctgtccaaaacatgggctcaggacagggtaatatctgggccatccctgggtcccatgcacaggtactggtctcaaaggtgctacccaaggcaggataaaactcagttccaaacctgagcctggactcctctcccctgaccttaagaacatgtcctcctgggtcccccgactgtggccagccaaaggctcatcccacgcctgactctccctgcacacatgtggctgctgcagaagagctgtcctttcaactccaggtggcgctgtacacccttactatcttgaagtccggtacacaggagggcgtgggctgaatcctctgccatccactagctgtgtagccttagaaaaggctaatcctgcccctaatcctgccacctcgatttcctcacttgtacacagtcaatagtaatccacacctcacagagtggagaggattcaagggatcagcaatgtgatgaggccagcacagtgcctggcactgagtgaggcttctgcaatgcagattccgtccttccctccaccctggggagagcatgaggccattgtcaagatgacccctgacacaaattggctagtccgagcccagagcgctgaagttcccagaaggaccgggagggggcgcccacccacattcttccccacctgagtctgcgctgacgatttcctgggcttatctggatcttcctgcagaaagtcagtcttatgtgaccctgtacaacctcctggactttcccgcgggcgtggtgcctgtcactatcgtgacactacaggacgaggaggaactggccttctacaaggggtgctacggagatagttctgacaaaaatttctcagaggtcagtttccttctccgagcctctcccggagcggggacaaaccagggctggttctctccgggttggggcccctgacggtagtggtggagagagtagggcgggactggtcattcctggtgttcaccctttggcacttatgctagtttcaccccaaccctgaggacacatcatttgacctccttgtcagccccatccatgtcaggggagaaaactttgcaaaaccagtggttttctttgtatttcttctgcctcctcctcctccccctccccctccccctcttcctccttctcctcctcctcttcctcctcctcctccttctccccctccttcttctttttcttcttctcctcctcctcctcctcctcctcctccttctccccctccttctccttctccttcttcctccttttccttctccttctccttctccttcttcctccttttccttctccttctccttcttttttgagacagagtcttgctctatcgcccaggctggagtgcagtggcacgatctcggctcactgcaacctctgcctcctgggttcaagtgattctcctgcctcagcctcccaagtagctgggattacaggcacctgccaccacgcccggctaatttttttttttttttttgagatggaatctcactcttttgcccaggctgatgtgcagtggtgcaatctcagctcactgcaacctccacatcctgagtttgagccatcctcctgcctctcagcctcccaagtagctgggactacaggcatgcaccaccatgctcggctaatttttgtaattttagtagagacacggtttcaccatgttggtcaggctggtctcaaactcctggcctcaagtgatctgcctgcctcggcctcccaatgtgctgggattacaggtgtgagccattgcgcccggccttctttgcattgctgtaggtaaaaatgatctcagaggcagggagggcagagcagggcaaaagccgctggttatgagcttactgtgtatctgctctggatatgacctctcttgggacctctgtttcttcaccaggaaaatgggaataaaaacatctactttgtagggttgtgctaaaggttaattaatttgaaaaagtgaatgaagcaatttgcataaggtcttgtgtgtaggaagtgttcgataaatactatgattagtaagtcagagtggtttcataaaagaaaatattaccaaatatttaactgcagggtctaaaataacacacctgactttggtgagagagagaaggagagagaggaagagaaagaggccgactctgaaacatatgcacgtatctgagtcagacattaagtaacttactttttctggaaattgattttagtgctagagttacccagtggaactgctgacctgaattctgagaaaataacaataatgacactatctcatgtgtcttgagcacttactctgttccaggagctgtttaaaagtgccgtgtataaatattaaatcattaaattcaataactctcctgtgaggttttttaaatgaggaaaatggaggcacagacagattaagggactgggccaaagccacacagccaattgaagtggaggagctaggacttgaaacaggtgatctgactccagagacaaaggcaaataaagcctcaaatgatatcatcacaaagcaaagaaaacaggtttgaattcctacaaggacgtttggatttcgtggcagggactcaggcttagcccccatgttcctgggcctgttttgggccaaggcaatgctttcactgtggaagggtaaccaggctctggatcagggattagcatgctcttctttctcttgcttgaacattgagtggatgctcggctttctctttcgtcattataatcagcattctgcacagggagcaagttttacatgttaaccctgaagaactatgggcaataaaatcagaacagtcttttcaggtttcactgagagctgaggaagcctggaattctgagatctaggtcatttttaccttaatatagattgggaaagggatgtttggactaaagcatacctagaccaaccgttggtacggaggcccagaatagcatgggtgatgaacagagccaggcaaggggcctgtgaagcaggctctgagttcccgaccttctctactggcaggcggtaagaggatccgtcggagttctggtgactgtgcagtgcattgctttgccatgggaagaggagctgtgtctccggttcatgaaggaggtggacaccttggtcaagaatcagagggggcccaagtgataggctcctggaatggagtaacagctcatgaaacacggggctggttgtggtggctcatacttgtaatcccagcagttcaggaggcagaggctggcagatcgcttgaggccacgagtttgagaccaacctgggcaacatagtgagaccctgcttctaaagcattttcttggtgttactcctgtagatcctcacccaagtgtgctcctgatgccccttccttctcatgaataccatgtccaccttatgtctcctccttctggaaccccaccaggttccttttctttgttggtccctctgtgtgggtgctcaatattcctcagatgggcccaggatggggagcagggtgaggagctcaataaacattttctgactggc

SEQ ID NO: 7 - DNA, 8131 bp, Homo sapiens
tttcgctcttgttgtgcaggctggagtgcaatggcgagatctcagctcactgcaacctctgcctaccggattcaagtgattctcctgcctcagcctcccgagtatctgggattacaggcgtgtgccaccatgcccagctaattttgtatttttagtagagatgggatttctccatgttagtcaggctggtcttgaactcctgacctcaggtgatctgcctgccttggcctcccaaagtgctgggattacaggcgtgagccactgtgcccggcctgccacagctttttgcctcgcttccctgggctccagactggacatctccaacaatctttcacatggcagttaggcaatctcatgcttaaaatctttggactcacttgtgccaagtccagaagccttgttatgacctgcaaggccatgattaacctgaccctgcagctggcccctgcggcctcatctcctgcccttcctcagtgctcacagcccggccacgtggcctgcaggtaatgttcagaacaccgagtgatctcccgcctccacgccctttgctcttggtgcttgctgtgcctggagtgttgttcctggggtctccacctaaagaccacctactcgtccaaggtgagggcaattgctcttccaactctgtcaggctgtgttgaaagagcttctttgtgcttctgcacgtggtcaaaagcaaggtctgtgtattaatagaacccaacatctgttaggctgtggagttgaatacccattatctcatttggaaagtgggcattactatttccatttaaaaaatttatttatttatttattttttgagacagagtctctctctgtcgcccaggctggagttcaatggcacgatcttggctcactgcaacctctgtctctgggttcaagtgattctcctgcctcagcctcccaagtagctgggattacaggcgcctgccactgtgcccggctatgttttgtatttgtagtagagatggggtttcaccacgttggccaggctggtttcgaactcccgacctcaggtggtccacctgccttggccaaagtgctgggattacaggcgtgagccactgcgcctggccttttttcttttctttttctttgagatggcgtcttcctctgccacccaggctggagtgcagtggtgcgatctcagctcactgcagcctccgcctcctggcttcaagcgattttcctgcctcagactcccgagtatagctgggactccaggcgcctgccaccatgcctggctatgttttgtatttgtggtagagatggggtttcactatgttggccaggctggtcctcaactcctgatctcaagtgatccgcccgccttggcctcccaaagtgctgagattacaggtgtgagctaccgtgtctggccctattatttccattttatacataaggaaactgaagttcagaggggattgctgacttgttgaaggctgatcattatgggttacagagaagacttgaaacccacacgctcaactctaaacttactgtgacttcctcatttgtacaatcatcacaagaacatgcattcaacattcttcggacaccagcctctgtgctaggcgaccacaacactttgaagacagaagcagtcctgtgtactgtgcacctctgccaatatctgtttacaggagatagctgccatgtccctgtccaccctcccttttctctcctggcgattgcgatattggagttttaggacacagccagagcacttgtcatttgttcctgttggacaccatttttaggattatcccaagagctctggctgtttctgctcttcctcccaacatgtgcttatccacaaatctgagcactggacctctgcaacttcatccaagtcacccataaacctatggatcacagcagaccaaggaaagggcgtgacctacacccttaacagacagacacataaccgagttttgagcttcccagccagatgtatctttagttcacatttctctggctgggcttagctgggccctcccaagtttcctacacatagatttggggtggcggccctgggcacctcaggaaggtgaagccacttgggatcgggctgtgtatgctcagcacccagcatggtgcctggtactcagtgggtacccagagaaggcttgttgaatggagcaatgggtgacttgttattagggaacccattttggtccattctgattacttcctcttctcacctccaatagggaattttccaatcagtccctgaccctttgctcctttcacatttattgtatctacctccatgatcttttttttttttttttttgagatggagtcttgcactgttgcccaggctggagtgcaatggcaggatctcggcttactgcaacctctgcctcctgggttcaagcgattttcctgcctcagcctccggagtagctgggattataggcgcctgccaccacgcccagctaattttttgtatttatagtagagatggggtttcactatgttggctaggctggtctcgaactcttgacctcaggcaatccacctgcctcagcctcccaaaatgctaggagccatgatcttgattagtgcccatgaggacaaataattcccagtctacattcaacctatagctttctcctggtctgtagatcctcatctatccacttctctcatcctcttaactccttcatctctctcaggctgttgaaagagcttctttgtgcttctgcacttggtagaaagcagggactgtgtcttaatagaatccaacatccgttaggctgtggagttgaacccattatctcctttgtaaaatgggcttattatttccatttcatatataaggaaactgaaattcagagagggttgctctctgaacaacaatggagggttgctccctccattcatcctcccatccatgcaataaaaatattgaattcttcccacagtatgttcagggtaaccaatcagaaatagtccctgcctgaatggagcttccattctaccaggaaacagacatcaaatgtagaattacacagaaacactcgttagaagtgcaatcaagcagaagccctgggtattatgagaataaaccacgtgggatctgatccagcctgagatgtgtgtatgtgtgtgtcagggaatgcttcctggaggaagtaacattgaagctgaaaactgcattgtcacctgagccaaggaatgagtgtgtttcaaggagggtgaagctgacaactctaaatgctgctgatttactcttgaggagatcactgggatgatataggcacaagccagactttgttgggtgggggagtgagtgaaaggtgaagaagtaaaggcagcccgtgtagaaaactggaaaagttcaggaagcggacaaaagacgtggtagtagttagggagggtgtaaatctgagggaatcatccctcatcccccaagataggagagacttagcatgttaaatgctgctaggaaagagctagcagcaacgcacagaggggggaagtcaaggtaggaatggagggctcaacctgccatcatttcttcactgaagagataccattgaacacataccatgtgccaggtgttttgaaaaaggctgacaaggtctatgctcccccaaccccccagctaatttttttgcattttctgtagagatggggtcttgccgtgttgtccaggttgagctcaaactcctgagctcaattgatccgcccaaagtgctgggattacaggcgtgagccactgtgcctggcctcgtctgtgcttttacggagcttattttctagggagggaggcaggaggtgagttacagatcaacaagaaaacttcagctaatgataagtgtaatgatgagataaaatgaggtatgtggtaacggaagggtgtaacccaggaaaaggtgaggtcacgaggcctagagtgctgtgccgtgggatgtggtgcgggtgacaagtggcctgggggagctgaagatatgggggagagctggagttcatgaaggtggagtgggggctatggaagaaaatggtcagaaaagaggcagaaggacagaggagggctggtctggaggccccagggagatgacagagtgttacagagtgggcaacttcagggtcacccttagtcaactgctgacctcgcatctgttcctttagaccctcgggtactcagactcaacattaccaaccatgaattcagttccttcccaccctaacctgctgctgccctggcttcctggtctggagggcaaaggcgccattctcctgggtacagtgacttgcagtctcagtgatgaccattgagatggagactggatggaggcccctgaggagagcagaatggttcccacatcagggcccctctgcaccacttttccagtctcctcatgtcttctctgttcctcgtctgggaagtcatctcccttacccccacaactcccctccaccagcagggagagtcaatagactggggaggctggaaccccggatcagagtcatggccttgctttggagtcaagggggaagcccagctgggcgggctggtctcatgtcctggcatcatctcccctggggtggatgcctgatgagccctgcccgctcctccaggtgttctttcctttcctctcttcctgtcccccagaacctccactctaggcaaacatggcctgttcagttccacctccatgcgtctgcttatgcggaacaaaggagctttgggagaatcctgaaggcaatgggaaccccaggagcaaccccatccataactcctgagggttggagtagggaatctgaggggtgggatctgagaggtaggatgggtgggagtaggatgtgacagaggtgaggtcagctgcccagctgcaggcttgggcccttcttcaggctcgcctgctaaagcctcttcctctgcatggcccgggagataggggttttgtcgccaggaagtccagatggggtaagaactaggaggaggttgatcactgccacacccagggcccgagatgtgcgtgggtgccctggcagcatcgctgacaaatactcctgaggaaacagcagctggattcacacaggtcgtgcaatacctaaggtggcttggctgtttgactccctgatgatgctacttctgctggccctgctgggggctggcctactgggggcttccctgctcacctcgtggcatgctccagcccggaacaagatccccagggcccagaagtggagggaggtagcactgcagaagatggaggacctggcccagtgactccggcagcaggtgagtcgacacgggtcccggaggcccccagccacagggggccttggccctcaatcccaacaggaggactacacctcaggatgcccctcccgtccatgaccccagcccccgcagacacagggagcaggtgggcacttccccacccccagttctccccccatgccagctctgtgtgtggttgtcagttctcctccatccccggcctttgagaccctggagattgggggcagtgtattctttctctgttctcccagcacttggcacgtggctcagtaacatgggaggtgcccacttagggtatttgcggaaataagataaactgatggaggccattggaggagggaggctcgatctcttttagcccctgagcactccaaaatcccccaagacaggaaccctagtctacctgtcccctcctacctccaccccattcagctctgaaaacacttgctgagccctgataagtgcagagcatggggggctggggatggggtctcccaggaagctgcaggtcttcagaggcagctttggcaactcggagtgggggtatttcactgggatagcctctgtggctggctgggctgagactggcaggcgaagtggctgagccatagatgtatcagcaaagcctgccccaggtggcagagagaagggcgggaaggagggacatggagacaaacatagactgagcctgggatttgctgtgtggcctggaggatgtgacaacccgtctctgggccttggactccccagctgtctgaggggggatgggctcatggtctctcggggtctccagctttggttgatgatggtggactcagtctgggagcccggaggtaggggctggggctagtgcctgaggtgctgttcccatgctttggagttcctgagtgtcctctgctgtcccctggatggtgattgatggccccaatgggcagcttctctgtctgagttgctgcagttgctgagtatgtgtattaatattaattagggctaattagttggataaatcaatctgcccccagagagcagctgcccctccctggttgatgaggaggaagtctgggctaatgggttgcagtggtgaatgggcatgatggaggcgtcctgtgtgcgtgtggaggccccatctgtgtgcggtggtgggtatagcttcctttactgcggacgagggcctgctttcttgtgcctcctgctggcatttcattgtgttgtggttggttgtgtgtctggtctggctgtgtggttatgtgcctggctgggtgtgcatgtgttgggttattggttggagtgtgtacatctagctatgtgtggctggtgtgggtctgaatgtctggtagagagtgtttgtgtgtggttgtgtgtctgatgtgtgggggcagctggtttggtatgtgtctgggcatctggttggtgaacatgtggatgtctgggctgttgggctggggacctggagggggtatatgtctggatggctggaggagtggaagaggttttggggtgaggtcactcatggtgtctccagcctcccattgtggtttcaggcttcttggctctcagcaccttgctgtctccccaacaagctatacaggtctgtcctgggcaccttctcagtcatgtcaccctctctctgccagtgacaacctcgagacctcaggtgtccacctttatgtcccggggaggtgcaaggctgggacacaggtcaaaccctcacaggctcagcaaacaaattcaattctgctgagtttagtaaaatttcccagggaatttctccaggtcttgccctgtgctgagctctggggacacattcattataaagatgaatctgacccctgactcacacttgtgctaaaaatgttcccaacctgggaggggcgtggtggagatagagctgtgcagactatgcagggcagcagcacggcagagtgtggtgaggccagatgcccacagaactggtgacttggcaggagggtggctggtctgtctggagaggatcatgttgggagggctccccagacgggtggtgagtgagctgaacctcatggcacctgtaggacttttctgaaaggagaaacgagaaaggcagtaccagggagggagaagccccagatgaggcagtgtttctgtagaacgtatagaaaataatattcctaggacccattgggtaaatggaccagctgctcatggctggaactgctcaagctactcatggccaggaagctctgctcacctcaggcagagcctggccaccttgagagttgacggtttttatgatactaaacatttaaccaccacattggaatttttttttttttcagacggagtctcactttgttgcccaggctggagtgcagtggcctgatctcagctccctgcaacctccacctcccgagttgaagcaattctcttgcctcagcctccagagtagctgggattacaggcaagtcccaccaagcccaactaatttttgtatttttcgtagacatggggtttcaccatgttggccaggatggtcttgatctcttgacctcgtgatcctcccaccttggcctcccaaagtgctgggattacaggcgtgagccaccgtgcccggccataaatattaataatacattgattcactaaaaactttaaattacattttttttgtttttcaaactaggctggaggcagcaccctgagtacagagaaggctggatgtccgtggggctgtgggatggagctggagggaagggttagctccaaactaaattacatattaaaaagtgatataacttgaggctcaatttttcatcaaattattcaaataatttgttgatttttagctttttttttttttttttggagacggag

SEQ ID NO: 8 - DNA, 22 bp, Artificial Sequence
  Primer sequence
ccaccagtgtgctggtggctac

SEQ ID NO: 9 - DNA, 22 bp, Artificial Sequence
  Primer sequence
agcctctggggcactttgactc

SEQ ID NO: 10 - DNA, 25 bp, Artificial Sequence
  Primer sequence
ttaatgtctggagtgataacatgac

SEQ ID NO: 11 - DNA, 25 bp, Artificial Sequence
  Primer sequence
acaacttctaattagtgttaatgac

SEQ ID NO: 12 - DNA, 22 bp, Artificial Sequence
  Primer sequence
aaggccgggcgcggtgacttac

SEQ ID NO: 13 - DNA, 23 bp, Artificial Sequence
  Primer sequence
ctctgggccatgttgctggttac

SEQ ID NO: 14 - DNA, 24 bp, Artificial Sequence
  Primer sequence
caactgtcacacaggccaaaacag

SEQ ID NO: 15 - DNA, 23 bp, Artificial Sequence
  Primer sequence
ccagaagtggagggaggtagcac

SEQ ID NO: 16 - DNA, 25 bp, Artificial Sequence
  Primer sequence
gctgtcataggtgtccttgaggctc

SEQ ID NO: 17 - DNA, 23 bp, Artificial Sequence
  Primer sequence
caaagtgagactccgtctgctgc

SEQ ID NO: 18 - DNA, 27 bp, Artificial Sequence
  Primer sequence
ggcaaaggcgccattctcctgggtaca

SEQ ID NO: 19 - DNA, 27 bp, Artificial Sequence
  Primer sequence
gccagtcagaaaatgtttattgagctc

SEQ ID NO: 20 - DNA, 23 bp, Artificial Sequence
  Primer sequence
actgacacaggtgacagcatctg

SEQ ID NO: 21 - DNA, 23 bp, Artificial Sequence
  Primer sequence
gtccagtcggtacatgtcttcac

SEQ ID NO: 22 - DNA, 18 bp, Artificial Sequence
  Primer sequence
cctggcacccagcacaat

SEQ ID NO: 23 - DNA, 19 bp, Artificial Sequence
  Primer sequence
gggccggactcgtcatact

SEQ ID NO: 24 - DNA, 21 bp, Artificial Sequence
  Guide sequence
cccagtgagtacgatggccag

SEQ ID NO: 25 - DNA, 21 bp, Artificial Sequence
  Guide sequence
ttagtgatattgttccgtggg

SEQ ID NO: 26 - DNA, 21 bp, Artificial Sequence
  Guide sequence
tcatggcctttccccttctca

SEQ ID NO: 27 - DNA, 21 bp, Artificial Sequence
  Guide sequence
gtcacttgcagtctgattaag

SEQ ID NO: 28 - DNA, 21 bp, Artificial Sequence
  Guide sequence 'FOP1'
aaaaggtgaggtcacgaggcc

SEQ ID NO: 29 - DNA, 57 bp, Homo sapiens
tttttttttttcgagacggagtttcgctcttgttgcccaggctggagtgcaatggca

SEQ ID NO: 30 - DNA, 298 bp, Homo sapiens
ttctttttttttttcgagacggagtttcgctcttgttgtgcaggctggagtgcaatggcgagatctcagctcactgcaacctctgcctaccggattcaagtgattctcctgcctcagcctcccgagtatctgggattacaggcgtgtgccaccatgcccagctaattttgtatttttagtagagatgggatttctccatgttagtcaggctggtcttgaactcctgacctcaggtgatctgcctgccttggcctcccaaagtgctgggattacaggcgtgagccactgtgcccggcct

SEQ ID NO: 31 - DNA, 295 bp, Homo sapiens
ttttttttttttttggagacggagtttcgctcttgttgcccaggctggagtgcaatggcatgatctcggctcaccgcaacctccgcctcccagattcaagcaattctcctatctcagcctcccaagtagctgggattacaggcatgtgccaccacgcccagctaattttgtatttttagtagagatggggtttctccatgttgaggctggtctcgaactcctgacctcaggtgatctgcccaccttcgcctcccaaagtgctgggattacaggcgtaagtcaccgcgcccggcct

SEQ ID NO: 32 - DNA, 560 bp, Homo sapiens
ggcctgctctatggcgtccctgtgagcctcaaggagtgcttcacctacaagggccaggactccacgctgggcttgagcctgaatgaaggggtgccggcggagtgcgacagcgtagtggtgcatgtgctgaagctgcagggtgccgtgcccttcgtgcacaccaatgttccacagtccatgttcagctatgactgcagtaaccccctctttggccagaccgtgaacccatggaagtcctccaaaagcccagggggctcctcagggggtgaaggggccctcatcgggtctggaggctcccccctgggcttaggcactgatatcggaggcagcatccgcttcccctcctccttctgcggcatctgcggcctcaagcccacagggaaccgcctcagcaagagtggcctgaagggctgtgtctatggacaggaggcagtgcgtctctccgtgggccccatggcccgggacgtggagagcctggcactgtgcctgcgagccctgctgtgcgaggacatgttccgcttggaccccactgtgcctcccttgcccttcagagaagaggt

SEQ ID NO: 33 - DNA, 561 bp, Homo sapiens
ggccttctctatggggtccccatgagcctcaaggacacctatgacagcatgggccatgactgtgcatgccgcctggcctagttcctggagaagcctgcgaccaaggacggggtcattatgaaagtgctcaaggcccaaggagccatcccctttgttaagaccaacatcccactgacgctgctcagctttgaatgcggcaactcccatctatggccagatgttgagcccactgaacttaaagaagacatgtgggggctcctcagggggtgaggggctctgctggcagaaagggggtccatcctaggcatgggtactgacacaggtgacagcatctgcataccagccagcttctgtggtgtttatggcctctggaccacaggttcccgcctcagctacactggaattgcctctgccatcaaggggaaaaaaatcggtgaccacggtggctggccccatggcccaggacgtggagagcctggcgctgtgcctgcaagccctgctgagtgaagacatgtaccgactggaccccactgtgctccagatgccctttagggaggaggt

SEQ ID NO: 34 - DNA, 221 bp, Homo sapiens
ctgtacaactgcctggacttccctgcaggggtggtgcctgtcaccacggtgactgctgaggacgaggcccagatggaacattacaggggctactttggggatatctgggacaagatgctgcagaagggcatgaagaagagtgtggggctgccggtggccgtgcagtgtgtggctctgccctggcaagaagagttgtgtctgcggttcatgcgggaggtgga

SEQ ID NO: 35 - DNA, 221 bp, Homo sapiens
ctgtacaacctcctggactttcccgcgggcgtggtgcctgtcactatcgtgacactacaggacgaggaggaactggccttctacaaggggtgctacggagatagttctgacaaaaatttctcagaggcggtaagaggatccgtcggacttctggtgactgtgcagtgcattgctttgccatgggaagaggagctgtgtctccggttcatgaaggaggtgga

SEQ ID NO: 36 - protein, 166 aa, Homo sapiens [sequence omitted]

SEQ ID NO: 37 - protein, 139 aa, Homo sapiens
SRSAGKLWELQHEIEVYRKTVIAQWRALDLDVVLTPMLAPALDLNAPGRATGAVSYTMLYNCLDFPAGVVPVTTVTAEDEAQMEHYRGYFGDIWDKMLQKGMKKSVGLPVAVQCVALPWQEELCLRFMREVERLMTPEK

SEQ ID NO: 38 - protein, 139 aa, Homo sapiens
SLTPKKLWEQHTAVEEYEQEFIAKWRSLDLDVLLVPVLGSAFYIGSSSLASESQSYVTLYNLLDFPAGVVPVTIVTLQDEEELAFYKGCYGDSSDKNFSEAVRGSVGLLVTVQCIALPWEEELCLRFMKEVDTLVKNQR

SEQ ID NO: 39 - DNA, 29582 bp, Homo sapiens
tctcctgcctcagcctcccaagtagctgggactacaggtgcctgccaccatgcccagctaatttttatatttttagtagagatggggtttcactgtgttagctaggatggtctcgatctcctgaccttgtgatccatctgccttggcctcccaaagtgctgggattacaggtgtgagccacctcacccggcctactttgacaatctttttaaaagtgtccttgtagactgcactggaagcaagccctattaggcattcgatttgcccagtttttcccttttccagagcctccaaagtccacttgcctgagggccatgactaaagtggtggcctcttttttatcctgtttgtcccattccacctgctcctcctgatctttattataaaaaaccaaggtttccaagttcaatagggtttctaagttttgctccaggcctaaggcggacttttgaagtttttttctaatgtctgcagctgactgagtgataaacttattcttcaagattagttggccttcaatagagttaggtgacagagaggtatgctttctcaatgcctcccttagtctctccagaaaggcagtaggattttcttcctttccctgtattatagtggacatcattgaataattcataggtttcttcctagttttccttagtccttctagcacgcaagttagcaaatgtctgctgcaccaatctccatgttctgattctgtgtcccagtgagggtctacactgggaactgcctgctggcctgtggggaatcgttctttcctctgttgtcatcttgtcattgacctgactgagataccagagatcaccaaactctcgggctgcagttatggcagcacttctctcatttgggtttagtgtctgatttagcaataacattatatctttccatgtcagatcaaaggattgtcctaacccttggaaaacatcaatatagccatcagggttatctgagaatttacctaggcctattttaatttgctttaagtctgagagagaaaaaggtacatgcactctggctgggccgaattctcctcctcccattgcttggagaggggcataattggggaatattagcactctttggttcattgtttacccctttgtctatctccttttggacgtttgggttgaaggggggtcctcattagttggggaaggagtcggggggacaccagggtagggaggtagactctagggcttcctgtaggacataaatcacactttttacataattgcgagttgtctcttaatgaaaagaaagtttgtacatatggcacttcattccatttgccttcttctctacaaaagaggtctcactgtaagatggtgttataatttatatttccctcaggaggccaggtttctcccccttgaagaggatatcatggccaggtggtactgcagaagaatataagtcatttctttcttagcgtctgagggtcaaattggtcccaaatctccagaatacatcttaggggcgtttttgccttgtggggaacgtttcccattgctttggaggtcccttcgtggtcgccaaatgttactggggggtccttgctcccagagctcccaagatggtggcgggccgcttccaagatggtggcaagcctggtgttctctgacctggggttcttggcctcacgaattccaaggaatggaatcttgggccatgcggtgagttttatagctctattagaagccgtgggtcatggaagagaactgtggaacccagtgactagtgttcagcttgattaggatgaacctgggcacttagccgtgcaggaacaatggcaaacctttagcctgattgggagcggcaatgggcgcctcgctggatcaggagcacagtagacaccctgccggatccagagggatggaagtcggcggcgggtctgcgatggcagcaaacagcagtggatgtcgagcgaaagctcagctccagccatagcaaacacggaccagaagagagtgcagttgcaagatttaatagagtgaaaacagagctcccatacaaagggaggggacccaaagagggtagccattttttcactttttttttttaacttttgttgaaaacattttaagtttggaatttcaactattctttgctattaataagacctcattcagtccatattaacttagaattggtatagatgggtccttcctgattctgtaagtgctttaaggcttggctgagtgcaaacagctctcacatttgaacaggccaattattaggcaattttcctaactctgcttctacaagagtttccttatcacttactgaatacccattgtgtctttttccctcaattacccaggaggaaccatctatcatcctgtcctgaagggagttcttcctaggtctggtcggacctttgtatggtaattaattaagatttagatcccatgttaggaaacctgctgggttaagggaattttcagtggttaatattaaatcatttttttctaacagaacagcctcatactttaaggttcttgagtcagtaagctacctttttttttttttgacttaggatagttctgacctgatgaggtgtgctcacaatgaggtttcctctaaaagttgtttttctactttcttctgttagcaaagcagttgctgctacagattgaatgcatttgggccatctgccggttactgggttaaggagttttgattagggaggttacgggttgtcagtggcctcagtgcttttgggctacatccttgtttacactgacaacaaggtggtattggagtgttatagggtcatggagaagaccttcaattatcaattacaggttttgaattttatcctggcttttaaaggaatagggtacactgttttctctttactacttctatctctctttctctctctctctctttgactctctctctctttccctgtctctgactccctctctctctctctttttcttttgagacagagtctagctctatcacccaggctggagtgcagtggcgcgatctcggctcactgcaagctccgcctcccaggttcacgccattctcctgcctcagcctcctgagtagctgggactacaggcgcccgccaccacgcctggctaatttttttgtatttttagtagagatggggtttcacggtgttagccaggatggtcttgatctcctgacctcgtgatccaccggccttggcctcccaaagtgctgggattacaggcatgagccaccacgcctggcttctgtctttctgtctctttctctctctgcctctctttctctctctttgcctctctctttctctccaacttcctctcccagtttctctttcctctctgctggtctttccctgcctctgccagctgcttatgctgctgttctcccctctccttccccttcccctagggaagggaccgtcaggagtgcagctactttttcttccccgagaagaaaggaaaggggaattctgaatatttttcttactaccggaggtttgtgtgaggtttttgatcccctgaaatttgtggaaggctcaacacctcaaaccagggggtatcttgccttgcctgacctggaaggctcaacccctcaaaccagggggtgttttgccttgctgccctggaaggctcaatccctcaaactaggaggtgtcttgccttgcttccctggaaggttgacctgtttcctccctttccccctctgaaggtcctttgcacacttcccactcgtgttgtcctctctggctgctcccccaagggagaattaggcccccctcagcattggcattccagtagaaatcccaccgcaggatcctccctaagccatatgaggtagctacggaaacgtggagaggacccactcactccgtccagcagtaggacttgtcatcatccacacgaacaacaccacaggtagggttgtttgtgatcattcacgcacacacacatttagccctccagaatttgaccaccaaggaagtaccttaccggctccctcggcttcttcctttgtctgtgcacagagttgtctctgcagtgtgtgaggatgctttaccctaggttgcctgctggtttcttttcacattgctgagagctcaggttatttcttgcactgggtgagtcctgatttctcacccctgaggccatcacaagagggtggggcatacctcctcaggagagagaaccagagactgcccctgaaggggaatgtaatcacgagcaagcccccaaattgttataaataaagtttccccccagtgccgcaaaagaaatagcactcgaatataaaattttcttttttttcttctcagcaaggcaatttacttctatagaagggtgcgccctcacagacggagcaaaggtgagcgcacacctggacaagggaggggaaggtggttcttatgcctgacccacgtgattcctgatgctgtgtccttcccctgttggctagggttagacctataggctaaactaattccgattggctaatttaaagacagtgagggggtgagtggtttggcgggaaaaatggttaccgcagagcaggaaatcggaatgaaccacggtgaagaatgagtgagggaggagcaggtaatcgaaaaatgttgctttatgaggaagttaagtttaaaagtagaaggcaaagaattgaagatactgacatattgattcttttaagataaatttagaactcatatctaacagctggcatgtctggcatggggctccggctggggcgcagtcttcagcatttggggctctggggtgcagggggcagaggacggccggggctgtggtgcccaaccggtgctaaactcaagcttgggaggtcgcccacgagaaacagtcgcccttccccacccgcctgctcggcttggcggggagcgggatgtcgctgggggcgatgccaggcgggccgcctctgatagcctctaggctctggcgcgcttccccgcccctcccgcgcaggcgggcgtgggatcccggctgatccagtccgggttttgcggcggagcgggcgggctgcgcgtgcggcggcttcaactgtcgcggtaggcagcagcaggctgaagggatcatggtgcagtacgagctgtgggccgcgctgcctggcgcctccggggtcgccctggcctgctgcttcgtggcggcggccgtggccctgcgctggtccgggcgccggacggcgcggggcgcggtggtccgggcgcgacagaggcagcgagcgggcctggagaacatggacagggcggcgcagcgcttccggctccaggtgactgccggagcgtagtgggatgggcgcggcctgagggtactcgcagcggcactttcagccgccggacccgccgagggacaggggatggggcgggcagagcagatgtgtaactctccagaatctctccttgccctaagatattccgcactttctgagccaggtagagcacgggggaagaaaggaaacggtagtgtcaaggcaggtggtggaaggcctttccctcactgggtcaaagaggagttttgctttgtgccaaagaatctcacgattgctgcctattggaatgcgaaaacgcaagcgtgacaaccagtgggatgccaggggttgaggactttggaatcgcagagtgtaatggccaaggggatctggagagcttagagttttgttttttgtttttttttgttttgttttgagacggagtctcgctctgactcccaggcaagagtgcagtggtgcgatctcggctcactgcaacctccgcctcccgggtgcaagcgattcttgctgcctcagcatccccagtagctgggattacaggggcccgccactacgcctggctaatttttgcatttttagtagagactgggtttcaccatgttggccaggctgatctcaaacgcctgacctcagttgatacacctgcctcggcctcccaaagtgctgggcgtgagccaccgcgcctggctgagttcaagcttcttgatttgtgcatttggatcctaagagggagccagaaagaaacctgccaagtgcacagggagatcttggcaaagccaggctagaagggaagtctctctggctcctgctgtggtgtccaacccctggcaagccctttccatgagcaggtttagttccagccctccgtgggtggtctgtcaacaagcttttctccctgcgctgcctttggatcacctcagtatgtgggtttggaggcgtggaagggcctggctgagggtttggaagatgtggcttgaagaggggcttttcctctgggtgtgtgaaacactgaccccagttaaagccttcttatgtgctgagagagggagggcttgctgtatctgtgggacctgacaggtgggaaggctttacaggttgggaaccgcaggactcaggagggtgtgcctgggtgggagacagaaagagtcacagaaaattgtgttcagcagatgttccgcaagtgatttttgagttggggcagagctggaactagaacctaggtgcccgctgcactctgcagccacactttcgtggagaggaacaggagagagatatgaggaaggcaccttgcatgccagcccagggtgtagccctgcatgttgaagggggccagcccctccacacctgtgggtatttctcctcaggtgggacaagagactgagaaaagaaataagacacagagacaaagtatagagaaagaacagtgggcccaggggaccaccgctcagtatagggaggacccgcgccagcactggtctctgagttccgtcagtatttattgatcactatctctaccatctcggtgagggggatgtggcaggactatagggtaatggtggggaaagggtcaacaggaaaacatgtgagcaaaggactctgtgtcataagtttaaggaaaggtgctgtgccttgatgtgtatgtaggccagatttatgtttgactttatacaagcatctcagtgcagtaaacaacagtattgtcaccagcatgtctcacctccagccataaggtggttttctcctatctcagtaaatagaacgtaggatcgggttttacactgacacattccattcccagggacgagcaggagatagatgccttcctcttatctcaactgcaaagaggccttcctctttcactgatcctcctcagcacagaccctttacgggtatcgggctgaggtatggtcaggtctttcccttcccacaaggccgtatctcaggctgtctcagtggggagaaaccttggagaatacccaggctttcttgggcagaggtgcctgcagccttccgcagtgcattgtgcccctgggtactcaagacgggagaatggcgatgactttttgccaagcatactgcctgcaaacacatttttaacaaagcacatcctgcacagccctaattaaaccttgagtcaacacagcacatgtttctgcgagcatagggttggggctaggtttacagattaccagcatctcaaggcagaagaatttctcttagtacagaacaaaatggaatttcttatgtctacttctttttacatagacacagtaacagtctgatctctcttttccccacacatgtgttgcggttttggctggctgtaatgtatgaatttactccaaaccatccctggggccaagatatctcatatttatttagtaagataaaaaatatatctggttccagcctccactcaccaagctggctgaaaagtccaccatcagtcagtttttagggtttcttccttccagagtgagagggccctggtggtcaacccaaattggccatctcccctacacaagcacaggttcttcactgtctagttgccctctctggctgggcgctggaggtcctccttagagatcctcctgtttatccctggctctgtgcagccagctgagttctgccagctccaagagcagcgtgggcagcactagcagggatctgctcacagctcttgcctgcagaactcccctcctggttgcaaggaatccacctggctggcaggggtgtgggatggtagcaggatgggtcttcctgcacttcggctccaaacagcagcatctatatggttttcctctggagcaactgctcttcattatttttacgaacagattattccaggacagaagttttggctctgaaagcttggctctttcaggaggagaagcgggaaattacctttcaggtttccagtgattgtggttttgagtaatcagcaaaggggtggggtcctgattgacaatagctttgtaggctttgcgggggagtaggatttttttttggtttttgttatttttgttttttgtttttgagacggagtcttgctctgtcgcccaggctggagtgcaatggtgcgatctcggcttactgcaacctctgcctcccaggttcaagcgattctcctgcctcagcctcccgagtagctgggattacaggcgcctgccaccatgcctggctaatttttgcatttttagtagagacggggcttcaccatgttggccatggctggcctcgacctcccgacctcaggtgatccgcccgcctcggcctcccaaagtgctgggattataggcatgagccaccgcgcctggccaatgcctggctaatttctgtagttttagtataaacggtttcgtcatgttggccaggctagtcttgaactctttttttttttttttttttgagatgaagtctcactttgttgccccagctggagtgcactggtgcaatctcggctcactgcaacctccacctcccgggttcaagcaattctcctgcctcagcctccctagtagctggggttacaggtgcctgccaccatgcccggctaatttttgtattttttagtagagatgggatttcaccatcttggccaggctggtcttgaactcctgacctcaggtgatccccctgccttggcttcccaaagtgttgggataacaggtgtgagccacctcacccggccaggacgtgggagttttagctgaacccagcccaggcttgggaacagctctttcccccgcctctcctcccttctgcctacaactcctaaggcacccttctgtttggctctggagtccttgaatgatgggcaggtaggatctgtgactgtctgggcaacctttcttctggggctcttagcccagccctgaatcacaagggggcacctgagataagcagggctccagcaggccctgggagaacacagcgatttgtagtaaagctcctgtctgatagattctggacaaagcgatttggcaaccaagattcttttttttttttgagtcagagtcttgctctgttgcccaggctggagtgtagtggctcaatcttggctcactgcaacctccgcctcccgggttcaagtgattctcctgcctcagcctcctggagtagctaggactacaggtgcctgccaccacatccagctaatttttgcatttttggtagagacagggtttcgccatgttggccaggctggtctcgaactcctgacctcaggtgatccgcctgcctcggcctcccaaagtgctgggattacaggtgtgagccaccactcccggattcttggctgtgtccaaggaggacacagctggatgaaggggtacctaaacaccttctgaattttcacaaaatagttcacctctctctaaactcttgagcaaatctagagaaaaatgtgtttctggtaattctgttgacgcttcacccattttttcccaccctgccccctgaataagttttgatatcttttctagaccgaagagaaggaccaccatcaatagaatagtatagctgggagagacatcacagaacacctatttatgcccttatgcctttgtacatgcagttttgttttaccctgaatggtttttcctacatctcttacaacccgcttatcaatcccactggcattgtggttcagaaggagaaaacaaaacagatggaggaggggcaatgcctcctaagtgattggtagagtatccctctcttgaaaaattgtgcatgcaggtggccacaggtttagatgttacctgtatactatacttccctgcattctccgcaaaatcaggtttccgcatgttcactgattggtcttctggaggtgcagacttactttggtgtctaggagaaaatgtctcagctgcctgacactagttgaagatttaaaaatagctgttagcagctgtgtcattaactgtcaacaggcaagaacataggaaagaatgaaaatgtgtgctgagcgtggaggggagcacattgctagctgctagctgccgtgcacaggcactctgtgggcgccttgtagcgaggtcgggggagttggtgaccggactgtcaggtggcagttattccagggtggtgaatgctctgctgatttcgatgtccttctccatactcttaggcattttttaaaatacaatgaacctgtatttatataatgaaaacaaaaataaagcaaaatttgattttcattgtgagatgggaaaggcaagatgcagtactgtgtgtatagtatgattcctttgtgcaaaaaagaatatatatagacaactgttgacatggtgggtttttcataaatattttcttttcctgtaagagtacaccagaaactgttaattatagttttcctttatagaggagggactgtgcaaggagaaccaggggtggagggaatgctcacttttcattttgtatacctttaaagaatatatcaagaggattatctagtgtgtttggggagaagtcttgaacccattttttcttctttgtagctccttgtgttagaaaaaaaatccaaagtaagtactctatcagttcaatgaattcagggaagtgctcctgacactgaggacatcagggggcagaggctgtggcatgtgctcggagagggcaggcgccaggctctggggtgtggggggtgggagggggcagtggtgcctgggtggggagaggtgcacatgagtctgagaggaccacagcttggaagcacctcctggaatatgctctggagcctgtggtgtgatgagatggggattttaaggggagaggcaaggccaggttgggttttgcactgtctggccctagtggaaagtgtgggttggaggtgcaggacctgggcagggcagcagttgggtggccgcgtgtgacctaggagacaaggatgagtctgaggcccggtgagggccttggtagaggggatggagaggtgaccatttttcagagctacttagcttggtgactggatgcaggtggtggtgggaaggaggagccagaaagacacctgtttcatttcctgaacacctggatggatggcggggcctcccctgagtacagggtacaggatacataaggaggagctggtcaaaagtcgggcaggtgatgagcttagaggaaggacagggaaggtggacaggtgacaggaatagcccagtgagctggtttgggctccattgcctcgggctgggtaggggatctgggggatgtgggatgagtggagagcctggagtcagaggtgcttaggggaggagtggaagccagggtaggggaggagggtaagaggggaggggaggaggggaagggtagaggggagaaggggaagcaaggggaggtgaggaagggaaggggagaagggaaaggaaggggaggggaggaagggaagggaagggtagagggggaggaggggaagcaaggggaggggaggaagggaagggtagagggggaggaggggaagccaggggaggggaggagggaaagggtagaggggaggagggaaaccaggggaggggaggaggggaaattggggagggaagagggggaagtggggaggggaggagggggaagcaggccaggggaggagggggagtagggggaggggagtagggggattagggggaggggaggagtagaagcagggttggaggggtgggaggaatggaagcaggaggaggggaagccttctcccagaatcagagagggaagagaaggtacccagagctctgtctctccccacatctggcatcttcttatccttcaaatcacagctgaaatgtggtttcttcagataggcagcctttaagaactggaacactcactgtgagggtctgcggcttcattcttgaagtcagtgagaccaagaacccaccaattccggacacagaatgaatgtgtaaacccttccttttgggtgtggccttcagtcacagacccagcctcccaagatggggtcttcttgtttttgcccttccctgctagaggttggcaaccccctgagtagtgttcagagctgctctgtgggtgtggggatggcatggggtcaggtgcaggcagatggctggtgggcaagaaggcacctctctctcagcctcagtttatctgtgcaatgggaatggcagtaagacttaatcaaaacatggatgacatcagcgtggtgttggcacacagaaggcagccactgctggtgtatatttgtagtggtttaatcatcagtctggagctaggcacagtagcatgtgcctgtagttccagctactcgggaggctgaagtgggaggatcacttgagcccaggagttcaagtctagcctgggcaacacggccagacactgtctctaaggaaaaaaaaaacctacttgggcaggtcggctcgctgggcaccccttcaacaagcttctggaggagacagagctgcattctctagggatggcaagggcctgcccaggctgggccatgtcagagctgctggggcatgggccactggtgtctgctgcaggcccatgagacttcggcgagtaggggactgatccgagtttgttccccacagaacccagacctggactcagaggcgctgctagccctgcccctgcctcagctggtgcagaagttacacagtagagagctggcccctgaggccgtgctcttcacctatgtgggaaaggtaaggccagccaaggccagcccctccctgggaaaggtaaggccagccaaggccagcccctccctttcccctccctctgtccgcacaggctgtggggaaaacctggcctggagttagtcctgctgggggccatggtgggacctacagtgccagggactgccagggagggaaggagccagagcgtgtgcgtgtgtgtatgtatgtgtgtatgagacactgagcatgctgtcttagctagtaacctggcttttagcccagacttccctctccctcctgcctccaccccattgggcaacaagtctggtctgttcccttctttttttttgagatggagtttcgctcttgttgttcaggctggagtgcaatggcacaatcttggcgcactgcaacctccacctcctgggttcaagcaattctcctgcctcagcctcccaagtagctgggattacaggcatgcaccactacacccggctaatgaaaagaaaaaaaattttttttttttttttgagatggagtctcgctctgttgcccaggctggaatgcagtggcatgatcttggctcactgcagcctccacctcctgggttcaagtgattcttctgcctcagcctcctgagtagctgggagtacaggcacctgctaacacacccagctaatttttgtatttttagtagagatgggattttaccatgttggtcaggctggtctggaactcctgacctcaagtgatccacccgcctcggtctcccaaagtgctggggttacagctgtgagccactgcagctggcccccaactaattttttgtatttagtagagacggggtttcaccatgttgatcaggctggtctcaaactcctgacctcaggtgatccacccgcctcggccttccaaagtgctaggattacaggcgtgagccaccatgcccgaccccgtctttttttttgagatgggagtcttgctctgtcgcccaggctggagtgcagtggcatgatcttggctcactacaacctccacctcccgggttcaagtgattctcatacctcagcctcccgagtagctgggattatagacatgcacccccatgcttggctaatttttgtatttttatttggccgggctggtctggaactcccaacctcaggtgatcctctgaaagtgctgggattacaggcgtgagccaccgcgcctggcctgttctcttcttttacccagccctctcctgtctccatcccctttggccaccctggcccgccaccaccatctcccgccatgcccaagcaccagcctcctggtcaggtgccctcttgtgtccccagctcttcaggccatctcttgtactcctcctctgtgtgtggcatcacctctggccaaggccttctggagcttgggtgtcagcagctctgcactggcttgggtggggctcctttacctggaaggctgtttccctcttctttgcccctgtccgtgccacgggctcccctggctgagccttcggggctcagagcaggaggcaccgtcttccattcgccacctgaggtagggtttcctcttccaggcctactctcattctaatagcacatttctcatcacagtgtcaggcttgtcttctctatctctttcccatggggggtctttgtggacagagcttgtctcatttgtctttgaaccttagtgctcaacatgttgcatttcacgtaataaatgctcaagaaatatgtttgaaaagaaagggagggagggaggaaagaaggagacaaattgtgctttgagtgtggcctgcatgatttcttgaaagggtgtgggacagtgagtgtgacccctaggcaggtgaacttgtctgggtgcagtgtatgtgacaatgctgtgggggctgcagctgaggaagcgagcgcatgctgggctggtgtcactgagagggggcacgtacatagtctcagcagatggtcttgcttcttccctgtcaatgtccctgaaaggctcctgcccttcctagttaatctagtctatctggttagattagccttctctgttcctgcctcgggtaccccggggacagattttgcacatgcctgaatatggcaacacagcccaccctgtttcccccagatactccccaggagcaggaatatttactgaaagctgcatctcactctgccctcacctttccttctgtaggaccctgtgtggtgaggtttgagcattctaggcagatttccactattagcatgttcttcccttttgtcaagctcctactccacatggcttgattatcaaattcaagatttcctgggtaaggggaggcttgactgggctacatgtggggaaggcgtggggttgaggagagactgctgggctccgggaggcaggagtctggtctagtcctgctctgtggttgcccttcagtgtgaccagtgatggggcgctgcccctgtctggtttctgtctgcctcactggcagagatgtggcttgggggaggtgagggagtggccagtggtcatcttcctcccagctcaccccctacctggggggcacctgaggccagtatcttgctcccttgagtgtcccggttgtgccctggtcctggttgaaggccagagacagccaggatgaggcctgggccaaatgtccctagtgaggcagatgctgagccctaggtcatcctctgtgccccaggctctgggccatgttgctggttacccctctccctgggtatactttaaaaggccagttctacatgatgtatatttcaccacaatttcttaaaaaggccagcctccttttatcttatgtctacttccccttcctcaggcctgggaagtgaacaaagggaccaactgtgtgacctcctatctggctgactgtgagactcagctgtctcaggccccaaggcagggcctgctctatggcgtccctgtgagcctcaaggagtgcttcacctacaaggtatgctctgcctcagcgccaggcctccatcgtcccctccatccctgccagcctgctctgcatcttgggtcattttgggcccttagaggaggtatcaggtccagaggccttccgaggggacactggtatacctgttttggcctgtgtgacagttgttggagtggacccttggctgcccacgggccctgactcactcccttctggtgcccatccctcctcccagggccaggactccacgctgggcttgagcctgaatgaaggggtgccggcggagtgcgacagcgtagtggtgcatgtgctgaagctgcagggtgccgtgcccttcgtgcacaccaatgttccacagtccatgttcaggttgggtcttggggtggggcggggcggggcaggggcaccggtcccagcatggcacgggctgacccattcttggctcctccagctatgactgcagtaaccccctctttggccagaccgtgaacccatggaagtcctccaaaagcccagggggctcctcagggggtgaaggggccctcatcgggtctggaggctcccccctgggcttaggcactgatatcggaggcagcatccgcttcccctcctccttctgcggcatctgcggcctcaagcccacagggaaccgcctcaggtaaggtgggtggagggcgcttctgggcccctcgctgtgtgaccttggcctagcttccaacctctctgggctccaggcggggattcggtctccggggttttgctgggaggaagcattacagtaccactggccgggcgtgggtcctagtttccaaagcggtgagtgttcagagctgctctgtgggtgtggggatggcggcgggtggccatttcctgtttccagcatcttatgtttcttatccagcaagagtggcctgaagggctgtgtctatggacaggaggcaggtgaggtccgtggtgctctcagtgccccgaggagggtgggggtcggcctgacccgcttccgcccgtgcttctcaggtggcagggcagtgtctggcccccaggctgctctaggtctgggttcctcgctccttgtctgcttacctccctcacctctctgccccacagtgcgtctctccgtgggccccatggcccgggacgtggagagcctggcactgtgcctgcgagccctgctgtgtgaggacatgttccgcttggaccccactgtgcctcccttgcccttcagagaagaggtgagcagggctgggtgggcatgaatgtggaccgctgaacccagacagccaccccaggccttgtgggcaggccttggagcccctgtctcctgagaaccgtcccccaggcctctgaggccagggcgggttgctcctccacagacggccaccagatggagcccttgcctgcatttggaaatcctcaggctttttttttttttccttttctttctttctttttttttttttttttgagactgagtatcgctctgtccctcaggctggagtgcagtggcgcgatctcggctcactgcaagctccgcctcccgggttcacgccattctcctgggttcacgccattctcctgcctcagcctcccgagtagctgggactacaggcgcccggcaccacgcccggctaattttttttgtatttttagtagtagagacggggtttcaccgtgttatccaggatggtctggatctcctgacctcgtgatccgcccgcctcggcctcccaaagtgctgggattacaggcttgagttaccgcgccggccggaaatccacaggctttcaaaggtgcccagcctcagctgctggcaccagggatgcaggaatcatttcccagcctgctgaccttcagcaaacagcagcctttctaacagtattcctgtccacattttgggagcagcacgccacgctgcctgcagaccccagctcatgtagcctgttcctgccagacttgctgctacgtgagccagggtctgcaagcagcgtggtgtgctgctccccaaaataccaccacagcagcctgttgctgagacaggctgggcttgttgctttctgtggcgaggcagcactgtcttgcaaagccttaggatcatctcagagggcaggaagggtggggagatctgctgagattttgaagtctggtttaaggtggatctttcaacatgggggttggttaagattggtttaagttggttaagattggttaagatccttaatccccatgttaaggattggtgggcacagcagggtgtggattttgaggcgagaggtgtcaaccgatgcttcctgttgaagagttggaatgaatcggaaggttatttgtgttatgtgtgttatttggaggaggtgggggagtggccagtggtcatcttcctcccagctcatcccctactgcggggcatctgagaccagtattttgctctcttgagtgttctggttgtgctctggtcctggtactctctctctctctgtctctgtgtgcgttggggttgaaggccagaaacagccaggttgaggctggggccagatgtccccagtgaggcaggtgctgggccctaggtcatcctctgtgcccactccaacagagtgcaggagctgtaaagttagattggtgcagacagaggaagagtgaagtcacgttaatgtagacagtaagctgtgtgacgtaagccccgtttctcagcagtccagcgattgtctatcttgtacagacctcttgccctcgccccagccaaggttgccttggaaaggctgagggtttgtggacgggaaggagagtgggccttggtgtttcttgggagtggggcagcagggcagatctgggctgggtagggtgaactccccctccccaggcagagggagatattctaaccgaacccacggggataggcagccgtgaagtccttcctcggaggagaggaggagatgaggtccctgtctggaagtctggaacagtttatcatgagagccaggacaggtggtggagagcctcagctcagaagacaggatgcctgcattccagacctgtcttgtcactctgcattgggtagctttgggcaagtcccagtcccacctaatctccctattgagacctcaagcctcagtttcctcatatgaccagtaggaatccttatccttgctctgcccacctgagtcactgtgaaggtgttttatgaaagggtcagatgcagaaggggctggcctcgctgactgcagcctcgcagctgtgtctggggctgagtagtttctctgatctctaggggtcctgcctagggttgtcttctcctgacctgcccctgtcccctgtgttttccctccaggtctacaccagctctcagcccctgcgtgtggggtactatgagactgacaactataccatgccctccccggccatgaggcgggccgtgctggagaccaaacagagccttgaggctgcggggcacacggtatgactgcagggtcctggaagtactggcatctcctcccctcacgggaagccttcctggtacccatggctactccatccctggcatcctggcactctgacgatgttgtcgtcggggtgaactgtgaccctgtgggacaagtatatagagggctgatcaagagtattggagtgagtgattgatggagaactttagccctgtgctgtgtgatgtgtgagcactgcatgtggggaggctcttcagctctaaacagtggtgcacagctgtccagaggctcccagggccagtgggttttggtctggtcattacacaactttatgtgtggctccagacttctctcatgctgtgcattccacagtgagttttcatgggtcagtaaggctgcctttgtagctctagtgagagctatcttgtgggcagggttggtccaatccatcctcagggccgcccagacagcatggggatcatgaagccagttgttaggtcaggaggccttacacccctcaatccctgcagctggttcccttcttgccaagcaacataccccatgctctggagaccctgtcaacaggtgggctcttcagtgatggtggccacaccttcctacagaacttgtgagtgatagtgggctttggggtcttggtgggatcagacaagtaggcagacctgggggagcagcagggtgtggtgatgcctggatgggccttagctgaatccaacaaaggcctgagcactctgggcagggacctcgctgtccctccagctgggcacattgagcctggagatcccttgccagggtgccagcccgaggggaggctgggttgagtatctgtggcctacccctgatctgagcttgttgtgaggtaggaggtgggcaggaggttgcctctctgtttgggaaggatttgggccaagggcaggatccaggcaggagggtgggggtttggacttgatgctgtgactccaggctctgtctgacttgagccaagtcttctttttgagcaggacctcagctttctctcctgtaaagtgggtgggttggaccagactccctttaagggactttgcagagctcatttttagagaagttcgttcctctgggatgcttctagtcattaaaggtgtcaggggcagagaacaggcctgcaaaggtgcctcctggtgacatacctctgctggatggactggaacccttcagaacacagtcccccttcctccacttcactgatggagaacttggccctgcagcctggagcttggccctgcagcttcactcagtcaagggcccagcctgtcatgttcctttccttcccctagcagccaagtgtggtccaggcttcagtggaaggggtcactcctcactctggccctgggaatgagtccccaggatcagctgcctgagacctttccctgagatcttgagccagagatagcctcagagccctgcttcatgggcagcccaccctcgatttccccacctgtgcctccaggctgtacctccctaaggggaggtaccctcagggaggcctcatcagggagatgttgccctcagttcttagagctctgagctgggtttgctggagagggataccctgagtcctgccttggggagctcccgtggatgtgggttgcagcccaggcatcccaaaggatcagcagaaacaaacggcatgtttggaaggagggagctgagtctggtgaggaggaggtggacaggatccctgcatagagaatgggattgctgtgggccgggcgagcaagctgggaaggatgtggggatgggagtgcctggaccgagcattttgtttcccagcaaaggtgatttcgtggacccctgcctgggggacctggtctcaattctgaagcttccccaatggcttaaaggactgctggccttcctggtgaagcctctggtgagggcacaaggagtggaggggctaggatggctgggggggaacctagggcctcctatcgcatgatcccccatggcctccctcagcctctcttggtttgggcaggcatggcctcctcttctctccagtccccacccagactgctctcctcctctgtcccctgcgatcttcagccaacccgcatgctgaaaggggtgccgacctgggccctggggggaggcatggagggaggggtccccagtggcttggcctgaagaaggttgacgtctgccgtggcccagagctgagtcaccgaccctgcgtctgtcctgtgcagctgccaaggctgtcagctttcctcagcaacatgaagtctcggtaagggttcttctgtgtctagctgccggcccctgcctgtcctgatccgagtctgggtctgggtagtttctgacaggaaaggacttgagggaagtagcctctgaggctggaagtggcccaggcaggggggcaacctttgtggccttcagatgggactttgaagttgtcttggcaaggtccagttctggctggagagcaaaggcctgagggggacaagaggatgggggagttggaggggaggaggttgacctggctggggcatgagtggaaaggaccaggaagtgggggttggcctgggccaagggtggggcacccgggagagatgccactgttagagatctgagctgacctgagctgcgccaggccctacttgccccttagtggctggggctggaaaagcagggcgtaaacctccctgtttcatgccctgacgtcccatggactcactccttcccttaccaccaggcttcaggactggcagcagctatggcctctcccgtgtcctgagggtagcgaggaatcgggcctgggctagtcctggctctgctgtggagtcaccaagtgccagcctgtgcccctctggggcctgattttctcatccagacagtaggggtttgaacttccctctcagagctcccatggggttgtgaagggtccacggaggggtgagatctagagggttggcagtaggggtctgatgttgctgatctccgtggctgtgaccatcatggctggtgaccacactccttctgcccagttcggctggaaaactctgggaactgcagcacgagatcgaggtgaggccagagcctctggattggagcagggtggtggggggagggtggagttggacagggtacccgctagcagtgtctcgtggccactgcccccatggggctcctagactggcctgtcatcccccttccactccctggaccaccacttgggcccagctctctgacccttacttgcctagatgcccatcctttgaggctgggtcagccccaggctcctgtcctggccgcctttttgcccctctggagctgcctttgtgtggctccgcctcagcgggaagaggtgtatccacaattcattctggaggcagaacgactgatgccctctgagaggcagcactgcctgcccggaggacctgtgtcccactgtggctctgttcagatccaggggcaggtgctggggccagagccaccccagccacagtccctgagttaaagagcctggggtgggctaggtctgagtgctttcacctggtgtgttgtgtcctccgcaggtgtaccgcaaaaccgtgattgcccagtggagggcgctggacctggatgtggtgctgacccccatgctggcccctgctctggacttgaatgccccaggcagggccacaggtgaggcccgacaccctgcctgtcccttctgtgaatctggccatgtgccctgcagggctgcgaggaaatggaagaagagccctctgggaggaccctgccctctcggggcccacagtctggctgactggagacatggcagtcatgtgggttgccctggcagggattgattttcctgtcatcagcactattcaagttggggatcttgagttacagaatctagtttggggaggtgatggtttgaagtccaggtgggatttagataaatcaagaaaataggggccagggcggtggctcacacctataatccgagcactttgggaggctgaggctggaggatcacttgagcccaggagctcaagagcagtccaggcaacatagtgaggctcctgttgctacaaaaaatagaaaaattagctgggtgtggttgcatgttcctgtagtcctggctactcggggggctgaggcaggaggattgcttgagcccaggaggtcaaggctgcagtgagttatgatcacaccactgcactccagcctgggtgacagagtgagactgtctcaaaaaaaggaaaaggaaaagaaaacaggaacagcattcccagtggagaaagtacatgggcaaaggcatggggcaaacatcagtgggttgtccagcccggccctgaaatctgaattcctgggctttgtcactcagacctcagtcctgggagagagcctttctctggctgtagacacagggtgccatttcatatgaggtttgactcaggcccggagttggcactgaagattctcagggcctgctgcagctgcctgtaatgtgttccaggggccgtcagctacactatgctgtacaactgcctggacttccctgcaggggtggtgcctgtcaccacggtgactgctgaggacgaggcccagatggaacattacaggggctactttggggatatctgggacaagatgctgcagaaggtgaggactgacctgcccctcaactggactcactccccaccctgactctggccgctgtggaggaaacagtaccagcactgcgggtttgccagcctttcttaagcaagacctgaaggactatggcctggccctacgttgtggcctctctctagctgggtgcttcctgggcctgggggtggggagtcctgccttgctaaccctatcctgatgcctgtatcccctatagggcatgaagaagagtgtggggctgccggtggccgtgcagtgtgtggctctgccctggcaagaagagttgtgtctgcggttcatgcgggaggtggagcgactgatgacccctgaaaagcagtcatcctgatggctctggctccagaggacctgagactcacactctctgcagcccagcctagtcagggcacagctgccctgctgccacagcaaggaaatgtcctgcatggggcagaggcttccgtgtcctctcccccaaccccctgcaagaagcgccgactccctgagtctggacctccatccctgctctggtcccctctcttcgtcctgatccctccacccccatgtggcagcccatgggtatgacataggccaaggcccaactaacagtcaagaaacagctcctcgtctgtgtggtttctgggcgtcatcgtgagggtggggtttggagcctgttgagagcagggctggcttgactgtgcatacccaggctccagccatgccagtctcctgctccacaacctcccctggtgcccatcacccacaggaggggtgcaggcttgtatcccccagcacttcggccgtgcccctcctctctcacctacactaagccctgctctgctggacactgcccttggtctccttccttcttctgcttctttccctgcctagaaagctctttctgttcctctgctttctatcctttgagacctgactcagatccttctctctccaggacacctttcctcctccctctgggccctggagtatatgggctatttcttcccagtctgccctgtgtggtgggcattggtgggtgtgtctgcctgccttagcacactggctttccttgacggcagggaacccattgccacatctctgtcttctgtggccagcacggcagcaggggaagcactgagttgggttgcagagagtccgaagtgctggccctgagctgctgctgtttgggagaggagcccatgggcctggggaggccggcatgagacaaggtgacctggtagagtgtgctctcagggctggccaaggcctggattgccctgggaaggtttcctgaaggaggtggacgtgtgttgagtctagaagttttccagagactgagctaggggttgaggacatctcagagagaagggacagtatgcccaaagatcagggtgggtttgctaaatggcaggcatgttgaatgggcacaggggaagcagagatataggtgaggacagatcaaggtggacttgggcagccaggtcaggaacttgagttctgtctcaaggacagtgggactctggaaagatcatagctcggcctgaggactagactcgtggggcaaaacctgtagaagggtaaagaagctgctccatgatccctaatttggggagaggggcctaaagcctgaaccttggcccaggggtaaagaggggccctttgggaattgacaggatggaggtgagctgtctcagctcgtctgctatccacctcttactggactatgtcacctggctggtagaaaggtggcatctgtagccgaccctaggagtttccttcttttttttttttttttagcagagtttcgctcttgttgctcaggctggtgtgcaatggtgtgatctcggctcactgcaactccgcctcctgggttcaagcaattttccacctcttgggttcaagtgattctcctgcctcagcctcctgagcagctgggattacaggcatgcgccaccatgcccggctaattttgtatttttagtagagacggggtttctccatgttggtcagactggtcttgaactcccgacctcaggtgatccgcccacctcggcctcccaaagtgctgggattacaggtgaaagccaccatgcccggctgaccctaggagtttcttaaccccattagcccagttgctttgctcttccctggccccagccctaattctcctgctggctggagatgtttcagagcctgagccctctaggtagggcaggtccacggctcctacctgtctgtctcagattctttctagaagagttgccttcccaagacttccttctccaccctggttttcatactcctccagaagtgctttgccctccaggttgccacacccattggcgcctgcaccatctcccagtgccatccctgcctctgtggggccattttcagggcagaggtgaggtcccaacctacatggggacacccagattgggacatctaggtagatgctgcactttgccctgatttcttgtaaccactgctgtaattttgcctttttcataaaaccactaccatctgccccagcttcctcctcctgccccatttctctctttcagttaccgatatctttgtgccttcagacacgaggctgcagagtggaggtgccttcactcgttcattgattcagcccttggagcctcagcatggccatgtccagacctcagctgacctgagtcaagcctgggcttctggggacgtggacattgacacaaacacatctgttcctcctgtgattagggctgggggacaggatagacaaggggtcaaatgctgccaaggggagggggaagtggtcactgaggctagtacatggccactgtgtttcatctccaccaccatgctctagtccaagccacctccctcatctggacgctgcagtgacttcccttctgggctccctgctttcaaccctggctgccctctaatccattctccacacagagctggaatgatcttttaaaagtataaatcaggctaggcgcagtggctcatgcctgtaatcctcgcactttgggaggctgaggcgggtggatcaccgaggtcaggagctccagactagcctggccaacatggcgaaaccctgtctctactaaaagtacaaaaagtcttgacaggcatggtggcgtgcatctgtagtcccagctactgaggaggcttggaacgtggctccaatgtcaccttccctgctcacccatttataaaacggcctcctttatttctttttctttttttgagacggagtctagttctgttgccaggctggagtgcagtggcgcgatctcagctcactgcaacctccacctcctgggttcaagcaattctcttgcctcagcctcctgaatagctgggattataggcaagcgacaccacgcccaggtagttttttttttttttttgagatagagtcttgctctgttgcccaggctggagtgcagtggcgcgatcttggctcgctgcaacctccctctgcctcccgggttcaagcgattctattgcctcagcctcctgagtagattgaattacaggcacgcgccaccatgcccaagctaatttttgtatttttagtagagacagggtttcaccatgtcaaccaggatggtcttgatctccttacctcgtgatctgcccgcctcggcctctcaaagtgctgggattacaggtatgagccaccacgcccggccttggtttcttgattatctcaagctgggccctgcttcagagctttcatgttagctcttctctctgcttggaacacgcagctccaatgtcaccttccctgctcacccatttataaaatggcctcccttgttactctcttttcttttttctttttttctttttttctgagacggagtcttgctctgttacccaggctggagtgcagtggcatgattttggcttactgcaacctctgcctcccggattcaaccaattctcctgccccagcctcccaagtagctgggattacaggtgtctgccaccatactcagcgaatttttgtatttttagttgggacggggtttcaacatgttggtctggctggtcttgagcttgtgatctgcctgcctgggcctcccaaagtgctgggattacaggggtaagccactgcacccgagcccttgtttctttctttcttttttttttttttgtttttttttgacagagtctcactctgtcgcccacgctggagtgcagtggcacaatttcagctcactgcaacctccgcctcctgggttcaagcggttctcctgcctcagcctcctgagtagctggtattacaggcgtgcgccaccacgcccagctaatttttgtattttagtagagatggggtttcaccatgttggtcaggctggcctcgaactcctgacctcatgatctgcctgcctgggccttacaggcatgagccaccacgccctgccccttgttactttctaataggttaccctttgttcttttttttttttttttttttattaagacggagttttgctcttgttgcccaggttggagtgtaatggcaggatcttggctcactgcaaactctgcctcctgggttcaagcaattctcctgcctcagcctcccaagtagctgggattacaggcatgcgccaccatgcccagctaattttgtatttttagtagagacagggtttctccatgttggtcaggctggtcttgaactcccgacctcaggtgatccaccctcctgggcctcccaaagtgctgggattacaggtgtgagccacctcgcctggccaccctttgttctttgtagcattatcactctctgagctctttgatgtttttttgtctcctccactaaaccataagcttcctgagagctgtgctttgtcttgttcatcacttgttcttggcttagaggatggtgctccacaaattctgggatgataaagtgtggctgtgtgaggggccaaggcactgtgctgggtgctggcagtgacaaatgaggcagccctggcccctgtcctcgtggagctcacattctggagggatttgttgaatgaacagaagggggacagagagttgtgctaatgaagacctctaaatatttaatgtctggagtgataacatgacttttgatccggaaaaaaggggaaagggaattctagaccacatttactgagtacctactatgagccatctactttctgggcacttcacagtcatgccatttaatcctctgtgaaccctatgatgggcatttttgccccccttttacagaaagtttacgtatcttgcccagggtcccacagctagaagttgggggcttggaaccgaaagctaggccagtctgtcagcaactgcatgaggtctttctgttgatgccaagccccagtgagtacgatggccagaagagtgagagcacaaatcagcctcctcctcatacctctctgaccaccagtgtgctggtggctactgcctgttttcatggcctttccccttctcaccgggtccactgccacagcttctttttttttttcgagacggagtttcgctcttgttgtgcaggctggagtgcaatggcgagatctcagctcactgcaacctctgcctaccggattcaagtgattctcctgcctcagcctcccgagtatc

SEQ ID NO: 40 - protein, 579 aa, Homo sapiens
MVQYELWAALPGASGVALACCFVAAAVALRWSGRRTARGAVVRARQRQRAGLENMDRAAQRFRLQNPDLDSEALLALPLPQLVQKLHSRELAPEAVLFTYVGKAWEVNKGTNCVTSYLADCETQLSQAPRQGLLYGVPVSLKECFTYKGQDSTLGLSLNEGVPAECDSVVVHVLKLQGAVPFVHTNVPQSMFSYDCSNPLFGQTVNPWKSSKSPGGSSGGEGALIGSGGSPLGLGTDIGGSIRFPSSFCGICGLKPTGNRLSKSGLKGCVYGQEAVRLSVGPMARDVESLALCLRALLCEDMFRLDPTVPPLPFREEVYTSSQPLRVGYYETDNYTMPSPAMRRAVLETKQSLEAAGHTLVPFLPSNIPHALETLSTGGLFSDGGHTFLQNFKGDFVDPCLGDLVSILKLPQWLKGLLAFLVKPLLPRLSAFLSNMKSRSAGKLWELQHEIEVYRKTVIAQWRALDLDVVLTPMLAPALDLNAPGRATGAVSYTMLYNCLDFPAGVVPVTTVTAEDEAQMEHYRGYFGDIWDKMLQKGMKKSVGLPVAVQCVALPWQEELCLRFMREVERLMTPEKQSS

SEQ ID NO: 41 - protein, 579 aa, Homo sapiens [sequence omitted]